European Patent Specification EP 4 281 035 B1, published July 9, 2025. Title: Skin Care Composition and Method of Using the Same. Applicant: The Procter & Gamble Company. The sequence listing filed with the application follows.

SEQUENCE LISTING (3 sequences)

SEQ ID NO: 1 - protein, 4 aa, Artificial Sequence
  Description of artificial sequence: acetyl tetrapeptide-11 (ac-PPYL)
PPYL

SEQ ID NO: 2 - DNA, 93231 bp, Homo sapiens
gtggacgcggcggccccgcggcgggggcagcgggcggcgggggcggaggcggccgctagcgccctgcccggcgccgcctccttcggcgttcgccccacggaccggcaggcggcggaccgcggcccaggtgcccgggggcgggcgggcgggcgggcgggaacgcgcgcgggggtccgcggtccgggcttcccaggtcccgggacccggagggcggcggacgggggaggggcaggggctgggcggcgcatgcgcggggcccggggtctcggggtctccgggtcccggggacccgggggcccggggtgcgcggctggggacctgagggcgaggagcgaggacacacaccgaggactcttgcgagggatctcggggcccagctcggcctccctcctagcgctgggggcctgcccggaacccgagtccgcggctgtccctggggtttggcgctgcgcggaggtcgggtctggggaccgcagcgactctgggtcttcgggttgtcccctcggagggagggcccacgggcggggacatcgggacttgccctttcctcggcgcagcggagctggggcgtcgccgactcagaaggtgctttccgagacctccagggatctccgaggcgaggaaacccgggccccggacagaccgaccctgggtgggtgcgcccggcttctgccgtcggacggagacgcgcgtgtttgttcctccagctgcgaccacctttgaggaacggttcccactttgtgccccaacgcggcggggcgaccccggacaggctgcgctgggccgggtggcttctctgcggaagccgcgccacgtcgctcccggtcggggccgctgagggtcgggcgcccaggtctttccggagtcccgggctgcgcggcccgcgtggtgcgggtgaagctggaggggcgcggggtggtgccagtggaagtcaggagggtcggccctgccccctcacgcaccccaaccgggcacaactgcacgcctgtgcttttctgaagtcttttttaaaagttaaaagagaggaagtgtgctccaagtgtcaggattctttccaagaaaaacccacagttgtccaatggcctgggcttcgtgggacctccggggctgcacgcccacgtcagcctcagccgacccctgccaggaaaccagggaggcccctcctctcccagcctccttgggataagggtgccttggggaactgggtcagggcaaggacacgggattttcctgggaaggaccctgcgacacccgtgtcgttgcggggcagggtcagcatgactttcctcttccaaggtgaagagttggggggcatccagagaacaaccgtaatcacttcctccttcaccttcttactgccaggctgaagctcagggccctgtctgctctgtggactcaacagtttgtggcaagacaagctcagaactgagaagctgtcaccacaggtaaatagaaggtttaatttactgtttccagatggaaatatttaagtgttttcagtgtttacttctgttgcactacagaccagcaatctgggggttattactttgtgatgcaaggttagatacgttttcagactgaaagtaaaatacatgtgcatggattcattttttttttttttttttttttttgagacggagtctcgctctgccgcccaggctggagtgcagtggcctaatctcagatcacagcaacctctgccactggggttcaagcgattctcttgcctcagcctcccgagtagctgggattacaggcgcctgccaccatgcccagctaatttttgtagttttagtagaggcggggtttcaccatcttggccaggctgatcttgaactcctgacctcatgatccacctgttcctcccaaagtgctgggattacagacgtgagccaccgtgcctggcctaggattcactttgaagttctgagttattgtgtgacttttgctaggaacttcattgcttcgtggcaggcatgttttgtataatttaaaacttgatgacattaactttgagaaacgtgagtgcttactagacccttgggatgtccacactgactggtaccgagtagtgtactgtctctgagctgttttcattttgatttgaatattaagcagatggcttcttgagatagacccgtgccagaacatgccagggataggctgaagaaacgggccagatgatacaaatttgtgtggtcaccatccatgagagaccagggacactggggctgatgatgacctctgcaactctgaagcaaaagtaaactaattggcaagttgggtgcggtggctcactcctgtaatcccagcactttggaagctggggtgggcagatcgcttgaggccaggagttcgagaccagcctggccaacatggtgaaaccttgtctctacaaaaaaatagaaatattgcctgggcatggtggcggacatctgtaatcccagctactcaagaaactgaggcaggagaatcgcttgagcctgggaggtgaaggttttagtgaactgagattgtgccactgcactgcagcctgggcgccagggcgagactccgtctcaaaaataaataaataaaataaaattaattaactaattgacattagaaaaaaatgttttttctttcttttcccacatcctttttttttttttttttttttttgtgacagagttttgctcttgtcacccaggctggagtgcagtggcatgatcttggctcaccgcaacgtccacctcacggattcgaacaatactcctgcctcagcctcccgagtagctgggattacaggcactcaccaccacacccggctaatttttgtatttttagtagaggtgggtttcaccatgttggctgggctggtctcaaactcctgacctcaggtgaaccgcctgccttggcctcccaaagggctgaggttacaggtgcgagccaccgcgccgggcccttttccgacatcttaaacgtaaagtaggagacgtgtcataatcatcgaatactgcagtggttttcattagctcctgtttgtcaaacttatgaacagagttttaaaaattgtgtatcagccgggtgcggtggctcacacctgtaatctttgggaggctgaggtgggcagatgacaagatcaggagtttgagaccagcctggccaatatggtgaaaccctgtctctactaaaaatacaaaaattagctgggcatggtggcgggtgcctatggtcccagctactcaggaggctgaagcaggagaatctcttgaacccgggaggtggaggttgcagtgagctgagatggcaccacagcaccccagcctgggtgacagagcaagactccgtttccaaaaaaaaaaaattgtatatgagagagacagaactagacagagaagaaggagaaaatgtgtcttctttatacactattttgtaacttgctttatcgagtaggttatgaaaaatcttcctatgtgaaaaacatttctgcatcatttgaaatgtctatataatatcccattgtgtttagatacaataatatttagccaatctctttatgtgtatatatttaatacagtcattctataaatattgactgagtagctgctgtgggctactgtccgcagtgctgaacaagacaagcatgaatccatgaaactgattttcataccagaatataaaaaagaaacttaaagataatcctcatcatggtaaaagatgaagaacctatttttgccgggacatcttactctttagtaattggtggccagtgttctttttcttgcatgctgttttggagagtctgttttttaaataaatatttaagtagcctgggcgcagtggctcacgcctatggtttcagcactttgtgaggccgaaggggatggattgcttgagcccagggcttcaagaccagcctgggcaacctggcgaaaccctgcatctactaaaaatacaaaaattagccaggtatagtggcgtgtgcctgtggccccatctacttgggaggctgaggtgggaggatcccttgagcctgagaagtggaggttgcagtgactgagatggcaccactacactccagcctgggtgacagagtgagacctggtctcaaaaaataaataaatatttatgtaatcatctttaagcagtgtttttaattttatttatttatttatttatttttgagacagggtctcactgtgtcacctaggctagagcacagctgcatgatcacggcctattgcagcctcgacctccctgggctcaggtgatcctcccacctcagcctcccaagcagctaggaccacaggcacacgccaccaggcctgactcatttttgtattttttgcagagacggggtcttgctatgttgttcagacctgtctcaaactcctgggctcaagccatcctcctgcctcggcctcccatagtgctgggactaagccatgaaccactgcacccggcataagtggtctttctttaaaaaaaaaaaaaaaaaaaaaaaaaaaaaaaaaaaaaaaccacattaattaaaatatgtatttgcttattataaatatatttgaaacatgccaatttttcttctctttttttgctctattggtttctgtgtgtggatggatatatttttaatggcaaataggatgagtgtctttacttccaagtagtcagtgtttttctttaatgtttgtactaattttgtcacattgcagttagaggttgtggcctgtctaatttctgcttttttggaacttgagagtctctgtttttatttgtttttggtagcctggcatagagtccatttttcttttcttttctttttttgagacggagtttagctcttgttgcccagactggcgtgcagtggcgcaatctcagctcactgcaacctccgcctcctgggttcaagcgattctcctgcctcagtctccccagtagctgggattacaggtgcccaccaccacacctggctattttttgtatttttagtagagacggggttttgccatgttggccaggctggtctcgaactcctgatctcaggtgatccacccgcctcggcctcccaaagtgctgggattacaggtgtgagccactgcgcccagctgtagatactttttaaaaaggtatagtttctgattatggggtagaaatgtgctatgtctgtcatttcagccttatgaattgcccagaataagctagatcacctttaaggccatgtggttagggaaacttgggcacagaatttacattttcaacttggtgataagatgggtttaaggtaagaatcaaataggagaaagccttagctgttccagcggcccatgtttaaaagaatgtgcttctttttccaagtatttctgccgcttgcatgcactgagcttctttggaaaggagcaccatgcaggcatattttccagacaggaccggatttgctcgttactcagaggtgtgtgcattctttgcttttaggatatttaattagcatcttttaatagtgatattacggtgtcttaaaagtttatgcatttgaaaagaaaagaacttactccttgccaggtctcaacctatcatggttatctttgcagctgagctgcgttggttttgaggctcacatatggtaaaagtggttggaaatctggaaatattgctgtgtatctgcaaagcagcttgatatagtggaaaaggtattaggtcattaatcatgagatttggattctagccccttagctgctgcctgccaggcctggagacctttgttctcttctttaaactgctgctttctcatcagaaaatgaagttcctctccataccacctctctgaagggctgtgaagctcgaagtggcagcttaaaaaactgcccatctcaggaggtgtcttaagaaggaggacataccgctggctcctgcctttctcacttagccaggtctgatacctgtgttgttttcactgtggccattttaggatttttcaaaggctttcagaaagcaacatgctaccgtaccccttatacaccaaaactggttttcattttggaatataaaagtgagatttctccaccagtacaataaagttgttacaagtggttcctatgtgtttgtttttgtttttgagacagagtctcactctgtcacccaggctgcagtgcagtggcacaatcttggctcactgcaacctccgcctcccgggttcaagcaattctcccacctcagcctcctaagtagctgggactacaggcacccgccaccacgcccagctaatttttgtatttttagtagagatggagtttcaccatgttggccaggctggttttgaacttctgacctcaggtgatccacctgcttcagcctcccaaagtcttaggattacaggcgtgagccaccacacccggcctcctgtgtgttttgaaggtgattgtgacctcaggttttggcagggctataccttgtgtttgctcttactccaactccatggcatacctggaccaggcctcttcatcttgaagagggatctgctgaaatgcaggcccagtgaatctccccatgcctggacacagttccgtcaagccaggacccggtgctgcctgcacccctgtttctgttagtctgactgtcctcgctgagtctaactccttgagggcagagaggatgtcttatttatttctgccccgctagccgtgtaaactgagtaggtacttgtaaatgttcattgaataagtacctgattaatagaatttaattcaagaagaatgtattgatgggcctgtgtggtcaccacagtactgagatgtaggtgggagctggctgaagggggaggcacctaaacaggagtgcagacagcggcacctacggatgatggcccgctccatcccaccgcagcgaaattgtcccagacctctgcagcttcccccacacctagactgagagagagctcttcttccttctgtagggagcaggtgtttcctccagatgtccaatatgtacctcccattacagcggtgttaggaaggtgagggctgccgctgaaagggtccccttcataatcatcactagatttggggtatattatggattaaatagaatttttataagatgacctgaggatctatttaaataaaatcctctttctttctgcaagatcatggatttaaattcaacacaactgacttcatagggaaggggtatggtgaaagggaagtgaggtgggcagcactgatatttaacaaggtgagggtccttctcctgctctgactgtcacattaaaatattcccaggagaaattggagaaaactcagatgaaatatcgtctgtgttccaggaggcaggactcatcggaatgcttttattttgctccattttaagagatttgcagataaagaggagtgaagatttctattcagatttacttgctttatattttaacttatagaccacaagccaactttcgaaagagcatcattttgaatagtaagagttaggaaggcaaatacagaaggactaatggcttccaagattatgagcttcataggaatggtttgagatgaggctatagtaaagcagaatattgaagttcccccaccccctttcatttttcatttttcatttttaagagtgagcgaggccaggcgtggaggctcacacctgtaatcccagcactttgggaggccgaggtgggcagatcacaaggtcaggagtttgagaccagcctggccatcatggtgaaaccctgtctctactaaatgtacaaaaattagccaggcttggtatcaggtgcctgtaatcccagctactcaggaggctgaggcaggaaaattgcttgaacccaggagtcggaggttgcagtgagctgagatcgcaccactgcacatctcagaaaaaaaaagagtgaggccccaagtttttttgcatttgtttgtaactgaatacgtctgaagttatgtgataaccacgccaaggtgacaaattgccaagtttcagtaaaagagacccagttatttagaggttgacacgtggatatgtccctttctaagaagttcgtggtcagctttacatgagtatttaaatgcgtgtttataattcagcaatatggcttgtaaaatacagattgccaatcaagtgacatgcaaatcttgatgatctgaaacaagttttcttctgttatctatggaagaaatggtaatagggatatttaagtgggatgaattttttgaagcattttcaggcagttttccacatggaacaaaataacattgagtgggctgctaacatgaggaacatattgccctctgcctaggattatgagtaaatttgataaattctagactgcagtctcattttagctcattttatgaggcagcttgacaactgggatagtgtctcttttttttgtcgggggtgttgaggctggagtctcgctctgctgcccaggctggagtgcactggcgtgatctcggctcactgcaacctctgcctccggggttccagtggttctcctacctcagcctcctgagaagctgggattgtaggcatgtgccaccacgcccggctaatttttgtattttttagtggagacgggctttcaccatgttggccaggctgggtctcaaactcctgacctgaagtgatctgcccgcctcagccaccctaagtactgggattacaggcatgagccaccacacctggcttctgttctatctgtgcattggggatgaaattaacacaaatgatgtttaaagaaaaaaatgctcagagaagttagaaatgtgctttaaattggaatcatctcttagtatgtaaaagttttttgtaatagaaacaagcagggcagtatttgacctgttgacagtgtccttggactttacaatttgtgaagcagcgtattttgcttgagttgtacgattgtcgtttttttccccccactttgacaactgttacagaacctgtcaccagatacaggcaagggaggttgggcttcccatctctgcacggcttccctgtgattcacaagcaagcaatcagaagtgcacaaaagtttagaacgcgattttcattctcttctttccttagaaaaactcgctttgttagccttttccagaaaggaaggcactcaattgttgtaatactcaaatcataaaaagaagcctagtctagtctattcagcaaggtgttctgaaagagggaattttttaagttcaattatgcgaagatcttgaaggtgggactcaaaggagagggctatcctgggaagaaggctttggaaaatgagaggcatgaaggggagagggtatttaaatgtgtttgaagccaaggatccttgagagaaaaagctggcactaacagcgttcaaagaacttgcgtgacaagtgatgactaatgacactgagggtgggttgtgggtgcctagtgaattcctccgaagccaagagagaggtttccagacccagggaagaaggtgtgtacacccagaagtagtgtagggacagagattccgatcacaagctgtgactggaagacgccgaccaccactgcagcagcctgaaaaccacagtcttgaaccgccagcgaagggctgggaagtgcggatccagggctggtgcactgaacccagaggagcaggctcccattcccagctaagggtggcagctggcggggatctttccagcagaaagctgtaagtggaagctttcaattcagagcagtagcaatgccttcaaagtcccaggcttcacgtgggaacagagaatgtgaagagtatttagcaggatgccaatataagaaatctatattggtgttcgtttgtttgtttttgagatggagtctcgctctgtcacccaggccggagtgcagtggtgcgatctcagctcactgcaatctctgcctcctgggttcaagcgattctcctgcctcagcctcctacatagctggtactacaggcacgcgccaccatgcctggctaaattgttgtatttttagtagagatggggtttcaccacgttggccaggctggtctcaaactcccggcctcatgatccgccctctgcagcctcccaaagtgctgggattacaggcgtgagccaccgcacctggcccaatattgtttgtttatttatttcttgacaggatctcactctgtcaccaggctggagtgcagtggtgtgatctcagctcactgcaacctccacctctctggctcaagcaatcctccctcctcagcctcctgagcagctgggactacaggtgcacaccaccacacccaactagattttgtgttttttgtagagatggggtttagccatgttcagctagtctcaaactcctgggctcaagtgatctgtccgccttggcctcccaaagtgttgggattacaggtgtgattcatgatgtccagcccagtatttttctttcactctggaaaccaaaaattattggctttttttcctgttgcattccctttacttagatgaatctagcaaggttggctgttagtgtctaggtcagaagtctaagtgaaagtgaatatttaaccacactcaagcacagctgatgatctttaatactaatagaggtataagacttaaaagaaacaagaacccagagggaaaatatggccatggactcagagaaaaccacggcagcttccatggactcataaaaagagctcaaaacctaggaagtggatggagactctttttggaatgaatgaattcaaatgtgggctttcttagtagattaaatcattttctagaaggaatttcagaaggatgtgtgcccaattatggtatcaggtctgttgtagactcttcaaggaggaagcctctgaaagacaagaaggaacaattaaaaattagaattcaggtgagtggatcacgaggtcaagagatcgagaccagcctggccaacatggtgaaaccccgtctctactaaaaatacaaaatttagctgggcatggtatggctgtagtcccagctactcgggaggctgaggcaggagaatcacttgaacccgggaggcggaggctgcagtgaaccaagattgtgccactgcactccagcctggcaacagcgagactccatctcaaaaataataagtaaataaataaataaataaaaattagaactcagaaaaggaattaatttcttctgagagagaaaaagatgagattctagcctaaggtgtaacacatccatccaccaggtatcatttttatacacgtgaagttaaatcaccaaaggaccaggtgagcagatgtggactttccgactgtgtgtgtgcgacttcctcagagccctcagtggcgttcccttttccgcgctagcgtttggtccctgcgcttttctggatgcccccaccccctctggctccacgaggccccctgtacgtcaccatcacctttgtgagcttgaaacctgtcacccacccgccttccagatgtcacctgggccctcccggaggccctcgccctcagtgtgtctgattctgagctgtcctgcgttttcccctcccctcaccctggcgacccttttcggtctcagttgccagcctcctgctagggctgggtgggggacatcaaaggcaggacaaggtgtagggtcctcacccaccacttagcagctctcagatgcagacagatttttcagctggcctgtggctcagtttccctcagctacaagaggggtgcatgctagggtttctctggattgctgcacctggcaggtagtgtgagcttggtaggtgcttccttgcttatcattgcctctcccatcttaatgttgtcccatccatccaatgtttatgggatgagaggttgataggagggcatggccctgacattccagggactgaccgacacgctgtctacacaaaccccttctggttcttctcgtgcactgggcgtgccggagacacactcccttaccctcataccccgccgcacccctgtgacctctacctttgagacctcagcttaaactcactcttagggaaggctccctgaaccacctgctggggttgtatgctgatgcaggtacttgtaacacctggtgcttttcctttcgtgcactcaggcagtgtttattcaagtgatggcttggtgacagtggctctccctgagaccccgtgaggccagagtccttggctcatcactcatggttgaacccggagcctcttgctggtaggtgcttcaggactggctctgggagcctgtggctcctgccgggtacccaccggttgagatacctcaagttttaaatgccacctccttcctgaagccttccttgctgctcccccaaactagaggcaggagttttgtccttcagataacctatggcatttgagtcactctgatttgatgaattctgccttcacttgagcagctattaggggcatatgtcagtcattcattcctcagttcatgtatttattcagcaaatatttactgagcacgtactgcgtgccaggcactgtcctgctgtggaaaacagcaggcatgattccctgccactaccaaccactgcatcgcataactggcagactcccagcttcaaggagaggcacggagggaaactgagagcagcctgcagaggggaaagagcggggacagagggtcacggaggtcgcaggggcgtgtgtgcagcacctgccagtgaacggaatgtgcggctccagatgtcgttgtctttaaacttcggaatttcctttcactaaagaaccaagtccagggggaggaaagagtgaatacaaattatccaagaaactcaagagctcattttagttctcctgattatgatcttaaaggcattaagcgctcaagttaaactccttgtgacccacataggttagcagaatttaaatcctaggtgattattaactctaatcatacatctaatgacctatattgaagatacactgcctgcttagttgtggcttcagcctttgctccgtcactgatagttctagcctgaaaagcaaatgagccctcatgctcacgatttcaccacagtcacataagcgggaagagcaggctcctggctgtggcgagcttgactccatttggtttgatagaaatgagaggtagatgattccctagacaaatgcaggcctttctcgaagcccctttcccaggacgacgtgacatgagtggtctgtgccttccagggcagccacgtcatgctttgcccagccagggcggtggggagggagacagccacatcctgcccggggctcctgggccccgctgcatcaagtgaaagcagggctggctccctgatgtccttggagaagtcgcccacactgctttcccccatgggagtgacaaggatgtgtcccgccagccttccacgacggaccccccactctctattaattcccaagaaaccaggccatggaggtgggtttgagggtttgtattggtgttttttaaagtcaggttgaccgagtgcggtggctcacgcttgtaatcccagcactttgggaggctgaggcgggcggatcacatgaggtcaggagttcaagaccagcctggccaacatggtgaaaccttgtctctactaaaactacaaaaaaaattacctgggcgtggtggtgggcgcctgtaatcccagctactcaggaggctgaggcaggagaaacccttgaactagggaggctgcagtgagccgagatcgcgccactccagcctgggtgacaagagtgagattctgcctcaaaataaataaagtcgggtttattaagatataatttacatacagtaattttttttttttttgagacagagtttcactcttgttgcccaggctggagtgcaatggcacgatctcagctcactgcaacctccgcttccagggttcaagccattctactgcctcagcctcctgagtagctgagattacaggtgtccaccaccatgccttgctaatttttgtatttttagtagagacaggttttcgctatgttggccaagctggtcttgaactcctgacctcaggtgatccgccagcctcggcctcccaaagtgctgggattacaggcatgagccactgcacccggccagtacatgctttcttgatttgtctgtttcccacctgtctcccctccctagaatggcagctccatgacgacagaggtgtttctctgttttctccatggctgcaccctcagctgctagaaggtggcccagcataggaggtatttaatgaagccttcctctccacttaaatctacacccttgtgcttattaaaaggtgacagttttctgtttgaaaattttattagtgttttaatgagaaagttattatttgggtaatgcctgaatatgaggaaaacattaagggtagaaatgtaattgttttcctatttcattcagtctatggattttattgaagattacagaattacttctttgtagctatggaagtaaaaaaataataagacgagtagctatttcaaaacgtagggctgataaatttgggatggtttgagaacgttaagttggggaactccatttctttttttacatttttatttattttcatttgtttatttatttatttgagacagagtttcgctctgttgcccaggctagagtgcaatgccatgatctcggctcactgcaacctctgcctccggggtataagtgattctcccatatcagcctcccgaggagctgggactacaggcgcctgccaccacacctggctaatttttgtatttttagtagagatgggatttggccatgtcagccaggctggcctcaaactcctgaccgcaggtgatccgcctgcccttggcctcccaaagtgctgggattacaggtgtgagccaccgcgcccagccagggaactgcatttctgacagtggctcagtagtttggaagttaactggcaaaggtggacagaatctttaaacatatgtggaggaattggagagtttacaagatagtgaagaactgccaggccatggtctggagaagatggaaacttgatgtttggggccattgtgtccctggggtgttggccaatttatgaaagaagcagttaagagcctgagtggcacttttgaggggctagaagggaagaccctggtaaacatcccaaactttggattgggacccaaaaaagctccatcccaggagtacaggtgacctggaaacggatcagcgtaatcgaggactgaagtccagttctagctacgcccagtccttgagactggattaaggtgatctcagattgcaaggacctcaaatgcctggcagaagcaagtgaatatccttctggaggaacagagcctcatcctaggcctctaattatttttaaggacaatttttcaaatgcaggctttcctccctttgcacagttcccttatgcataaatttcagtcagtggccagctgcagtggctcatgcatgtaatcccagcgctttgggaggccaaggcgggtgaattgcttgagtctgggagttggagaccggcctgggcaacatagaaccccatctctatttttaaaaataaaatattaattatcactgcttagttaaattatagtggtctcccaacaatacagatcagatcccagctcccatggtatatacactgtgagtgctgtataaagtacaagctctgccgccagttctccagcctacaaatcacagtatagataacagatgtgcatgatgatcactggccaattgcgtcacttctctcaaagtcagtctgtgattggtccctgagcatctgtcggtcagtttcatgcacagactgcaaagcatatggttttgtctactctttgtctctcagtgataaacccacatggcattttgtaaaagtggatacatcaggccaggtgtggtggctcatgcctgtaatcccagcactttgggaggctgaggcaggtggatcatttggggtcaggagtttgagaccagcctggccaacatggtgaaaccccatctctactaaaaatacaaaaattagctggatgtggtggcaggcgcctgtaatcccagttactggggaggctgaggcaggagaattgcttgaacccaggaggcagagcttgcagtgagccgagatcatgccactgcactctagcctgggtgacagagcaagactaccatctcaaaaaaaaaaaaacaaaaaacagtaatcaagcatgaaaattatgaaatgctcagagataaaatgcgcgaggcctgtacactgtaatctacaaaacactgctgagagaaattttaaaagacctaaataaatggcaagttataacatgctcttgaatcagaagactcagtatcttaggatggcgacttttcccaaaatgatctacagattcaaagcaatcggaatcagacctcagcatgcctacttgtagaatttgataacctgattctaaagtttatatggaaatgcaaggaacccagagttgctaaaataactttgaaaaagaacaacacagttgaaggacttagactacatgatttcaagaattattataaagctacagtaatcaagacagtatggtattgatatgaaaatagaccattagatgaatggaacagaatagcaagtccagaaatagatccacacatatatggtcaattgattttcagcaaagtgccaagtcatttaagtggggaaaagataatcttttcaacaaatgataccggaacaactggatagccatatgcaaaagaacctcaaccttcagctcacagcactacaaactcataattattatcattatattatactattatgtaataatagtatatatcatgttacatattatattatgtaatatatattatatgatactgttatgtcatataattattattgaaatgggtcatagatctaattgtaagagttaaaaccatccaggtacagtggctcatgcctgtcatcttgcactttgagaggccaaggcgggtggatcacttggccccaggagttacaagaccatcctgggcaacatagcgaaacaccgtctctacaaaaaaatgaaaaaattagttgagcatgatgacactcacctgtagtcccagctgcacagtagtctgaggtgggaggatcacctgagcccagagaggtcaaggttgcagtgagccatgattgcaccactgcactccagactgggtgacagagagaccgtgtgttaaaaaaagagttaaaactataaaaccttcagaagaaaacatatgagaaaattctagtgatttggggtttggcaaagattccttgaacatgatttaaaaagcattaactaggccaggtatgctggcttacacctgtcattccaatgctttgggggaccgaggtgagaggatagcttgaggccaggagtccgagagcagcctgggcaacataacaagagtgggtctttaccaaaaaaaaaaaataaaaagcctgtgccaggcacagtggcacatgtctgtagtcctagctactcacgaagctgaggcaggaggatcacttgagcccaggagttgaagcttgcagtgaattatgaccatgccactgcactccagcctgggccacagagtaagactaagactcagtctcttaaagaagaaagcgaccgggcgcagtggctcacgcctgtaatcccagcactttgggaggctgaagcaggtggatcacaagggcaggagatgaagaccatcctggctaacacggtgaaaccccatctctactaaaaatacaaaaaattagccggacgtggtggtaggcgcctgtagtcctagctactcgggaggctgaggcaggagaatggcgtgaacctgggaggcggagcttgcagtgagccaagatcgtaccactgcactccagcctggacaacagagcgagactccatctcaaaaaaaaaaaaaaaaaaaaaaaaaaagaagaaagcataaactataaaagaaaaaattaataaattagtcatcctcaaaattagaaacttttactcatcagaaaacacttaataaaatgaaaagtcaagccatagacttagagaaaatatttacaaaacatatatctgacaaaggacttggatatggattatataaagaactattgtaattcaataagatgtcaaacaacccaattaaaaatgggtgaaagatgaactaactcttcaacaatgggcatgtcatttgaatggatggtaagcaagcacatgaaaagatgttcatgtgcctttccctcattagtcactagggaaatgcaagttcatagacatctctcttcgtagaaagatatcactacacacccacaagagtggctgtaattaagcagtctgaccaagtatgcgtaagaatgtggaataagaactctcatacactgctgatgggaatgtaaaatgatagccactttggaaaacattttggcaaataataccacttacattattatcgaaaatattgtatacctgaaagaactcaaagtgaaaaagctatatactgtctgcttccaaggctacacattatgggaaaggcaaaactatgaagacagtaaaaagatgcgccagtggttgccaggggctcatggggagggaaagaggaatgaataggtggaacacagggcatgtttagggcagtgaaactattctgtatggtaccgtaacgatgaatacatgttattaggcatttgtcaatacccataaaatgtacaacacaaagagtgaaaatgaaaactgtgggcttcagttagcaataatatgtcaacattggctcatcagtggcaacaaatgtacctcaccaatgcaagatgtttgtttgttgtttgtttgttttgtgacggagggggtgcagtggcgcaatctcggctcactgcaagctccgcctcccgggttcacgccaatctcctgcttcagcctccggagtagctgggactacaggcgcccgccaccacgcccggctaattttttgtatttttagtagagacggggtttcaccatgctagccaggatggtcttgatctcctgctgtcgtgatctgcccgcctcggcctcccaaagtgctgggattacaggcatgagccatcacgcccggccaccaatgcaagatgttaataacagggaaactgtggtgggagtgaggtggtatatgagacctctctgtactttccactcaatttttctgtaagcccaaaacttctctaaataagaaagtttattaattaaaagttacttttatagtgtatctatatctaggaataaatctgaaaaagatatataagatctctactcagaaaactgattatgttattaagagagcttaaatatagcccaaataaatagatggatatactatgttcatggaagggacagctcagtattaggaaggtgtcagtcatcttaagaaaagcctcatgtgtcacacaagggatactgacatctgacaccaagcacatgtaggcatcctgactacgtttacttgaatgatgtggactttacagagctgactatagacagttcaaatggcctgaaaactgttcaatgcactccctcccaggctgtcatgggatgcacttcaggaactttactttttaacaagaaaattcagttttcctcttaaacagctggcttctgttccattagcattcttgtcactttaagttgcattcatctttgttttttttttttagaaaaacatttgttctgcaaccagtcttgtcctttaaatacttgtactgtatacaggctctttttcataggtccattacttaaaatgatgtaagtgtgtttttggtggcaggggggtgggagttgtttgttttgttttgttgagacacggtcttactctgtcacccaggctggagtgcagtggtgtgatcttggctcactcctggcctcaagtgatccacccacctcagcctcctaagtagctgggaccacaggtgtgtaccaccacacccagctaatttttttttttttttttttttttttttgtagggacggggttttgtcatatcacccaggctggtctcaaactcctggactcaagggatcagcctgtctcagcctcccaaagtgctgggattacaggtgtgagccactgcaccggtcctgatttgagtttttgtaagacagggaacaatgttcagaatttagcaccaatgtcagactcattctgtaaatttttattgaacgtctgcctggtgtaggagaggaagatgacagacaagaattcttcctccaagagttacaggtcagttgagcagaaaaggcatacatcaatacccacaatgagagttgtcgtgattcagaggagggacaaagtccttcccctggagggatcctgagcactttggagaggaaaggcatctgtactgccccccaaatgtgtagaatgggatgcattcctggcagaaagaagtaggataaagtacagaggccagggctgggtgcagtggttcacgcctgtaatcccagcactttgggaggccgagacagcagatcacctgaggtcaggagttcgagaccagcctggtcaacatggcaaaaccctctctctactaaaaatacaaaaattagccaggcacaatggcaggtacctgtaatcccagctacttgggaggctgaggcaggagaattgcttgagcccaggaggcagagatcgcagtgagccaagactgcgccactgcactccagcctgggcaacagagcaagactctgtctcataaaaaaagaaaaaaaaaaagtacagagtccaggaagcctggggtggggctggcagatgccgagtcatctattttggccagagttcaaggcttgctaggggacatgaagagaagattcgtgcattctagttcaaactccaccagatatttgagctccttctctgtaccaggcattgttctaagatacgtaagtgaacaaaacccatgacaccctcgtctatgagagctgatcctctggcagggacagacaggtcatgagtggagtgatggagcagctggcctggtgacttagccgccttcaggtacagtaggaggagcaagcccaggacaggtgagtgggtcaagggtgccagaaggggtgagggcaccaggaagctggtccagtttggcttccctgaggtggtgaccaggacctagcatctgaggaagggctggaagcaggtgagagcaggtggagcagacatcaggatgggagcatcctgacagggagggcagcagggtgggctcatgagaggaacagccaggaagtgtgactcgagcagtgtcctggagaggaggaggaggagaaagaggtcaggaggtcccaggggagaggcaggaccagtctcgtggaggtcggggccgttgtgaggactctggtttgtgttgtgtgtgaaaggccatgggatggggaccagcgagggcttcttaggggactggatatgctctgatctagctgctaaaaagcccccttgggcagcttgcagggcccgggcagaagctataggtggttctgaggtttgcagaggggcctgaaggggtggggcccggccaagcaaggtggctaagtgggaaaggctccaccgcgttgggtgtaggaagaccttgaccttagctccagcccagccactgagcagccgtgtcgccttgggtgatacctgtccctggtcggtttccctacctgtgaatctgggtacttggaagccatgctcgagaagagcccatccccaggaggtgatcagggttctccttcaggtgaggaacctggcagccgtgtgtgagaaccttagaaaagggagagggaagaggctgtggcaggaagtgaggagggagttagtgataccctgggcaggatgccatgagctgggatggaaaccacaggatgaatgcaagtaattaaaaaaaaaaaaaaaaaaaaaacagcattgggccgggcagtggctcacgcctgtaatcccagcattttgggaggccgaggtaggtggatcacctgaagtcaggagttggagaccagcctagccaacatggtgaaactgaaaatgcaaaaattagccaggcatggtggcgtgtgactatagttccagctactcaggaggctgagacaggagaatcacttgaacctgggaggtggatgttgctgtgagctgagatcgtgccactgcattgcagcctcggtgagagagcaaggccccatctcaaaaaagaaaaaaacagactttccgaccaaacgatcgacaaaccagactgtccaaacagccataagccgtaactttgtgcggaggtaaaagaccgaggtcacatcgggacctgttggattcaaggcatgttgacagctgtttccaggcttcagatagagcctccagctggcagggtggccacagggcttgttgagtaggaagcctcgttgctttgacaggttacttggccccatgagggacaatcccatagtcagttacccagaaacgtgactgtctccttgaaatcctcagcatggggtcttatgaataaacccttactagatttcctgttctgtcttatttttatgcagagctttactttatagcagaaaattccatttttacccttaaatggcttgcttctgctcccttagtgttcttgtcactttaagttgcattcatctttgtccctttagaaaaggatttgtcctgcaaccagctcttgcagaaggtacttggtttattgttaaccgatgtttgctaaatgtttgaattatgttgagttgcttaaagtcatgctatcgggtagatgttgtggctgttcttttcactctcttatttggggatttacaaaacagttatgtttttagttttcttttatttgttgtgttgaataggaatgtagctctgggaacctctagttccaaataagaaagccttggacacatttccagttggcaagctggcaaaatgaagggcgtacaagttgttagagaggctgggagcctatttaagcacccagcttcaggatgggacatgggatatacctcgagttagaggttcttattaactgtggattcttctatgcagatatctgtcacaatataagttactataagtcagtactaaggcagctgctacattctgtttgccaaggggaagaagaaagcttggaaatggtattccttaaaaatgtcagtatcataaaagacaaagaaaagctgcggaaatgtttcagattaaaagagagaagacaataaaatgtaatacctgactctgaacagcatccagtactgaaggaggaaaaatgctatcaaggacattattgggtcaattaacaaaatttgaatacgaatcatagattgaactgtatctgttaaattaacagaagcgaagtgttctgtggtgtgtaggagcacactgccattcttagcaaacgtgtagtttagtatttaggagaaagggccatgaggcatgcaactcaccctcaaatacacacacacatacacatatatacatacatacctataaagaaagaaattatgggctaggtgcagtggctcatgcctgtaatcccagcactttgggaggccgaggtgggtggattgtgaggtcaggagatcgagaccctctctactaaaatacaaagaattagctgggcgtggtggtgcacgtctgtagtcccagctactcgggaggctgaggcaggagaattgcttgaacccaggaggcagaggttacagtgagccgagattgcaccactgcactgcagcctggcaacagagcaagactctgtcttgaaagaaggaagaaagagagagagagagagagagagagagagggagaaagaaagagagagagaaagaaagaaagaaggaaggaaggaaggaaggaaggaaattatgataaagcagatggttaagttggtaactaccagtgaatatgggtaaagttaggatgttctttactctgttttgggggtgcaacttttctataagtgaaagtacttccaaataaaaagttaaaaggcaagcaaataaataaaagagacagtttctatgttatatatcctagctatgtttaccatgtctggattctgaaagctgcagagcagaaaacctgaagaacagatcacctgttcttaaaataccactgttggccagacatagtaactcactcctgtaatcccagcactttgggaagccgaggtgggaggatcacctgagctcaggagtttgagaacagcctgggaaacatagtgagaccctgtctctacaaaaatttaaaaaattatccaggcatcatggttcgtgcctgtagtcctagctactcaggaggctgaggtaggaggattgcttgagcctgggagttcgaggctgcagtgaaccatgatcacactaaagcactctagcctgggcaacagagcaagaccctgtatcaaaaaaacaatcaaacaaaaaatcactcctaattttcctcccttttagtacttttaaaaattaacttaaaacattttttggataattgtagttttttttacttttttttttttgagacagagtctcattctgtcacccaggctggagtgtactggtgcaatctcaggtgactgcaacctctgtctcctggattcaagtgattctcctgcctcagcctcctgagtagctgggttcataggcgtgcaccacacctggctcgtttttatatttttagtagagatggggtttcaccttgttggccaggctggtctcagattcctgacttcaagtgatctgcccgccttggcctcacgtgcagttttaggaaataatacagagatccccagcactctttccagttttccccaagggtaacatcttgcaaagtgagaggacgatatcacagtcaggatactgacattgataccatcaagatacataatgtttccatcaccaatcagtggtcatggtgccttttatagccaaacccacttctctcctaccttcccatcccttttttaattttgccagtcattaatctgttgcccatttctgtcattttatgaatgtcacataggccgggcgcggtggctcacgcctgtaatcccagcactttgggaggccgaggcaggcggatcacgaggtcaggagatcgagaccatcctggctaacatggtgaaaccccatctctactaaaaaatacaaaaaattagccaagcgtggtggcgggcgcctgtagtcccagctactcgggaggctgaggcaggagaatggtgtggacccgggagacggagcttgtagtgagctgaaatcacaccactgcactccagactgggtgacaaagcgagactccatcttaaaaaaaaaaaaaaaagaatgtcacataatgaatcatatggcatataaccgtttgagactcagggtaattctcatgagactcatccagcttgttggtgcatcaacagtttattcctttttattgctgagtaatttccatggtatggaggaaccatggtttaactattcacccattggaggacatctaggttgtttccagcttggagttattatgaataaagctgctgtgaacatttgtgtacaggtttcttggttttctggtttgttttaaacagttctagccaggcacggtggctcacacctgtaatcctaacacttggaaggctgaggtaggaggactgcttgatcctaggaggcagaggttgcaaggagccgaaattgtgccactgtactccagcctgggcaacatagcaagaccctgtcattcataggtaggtggatggatggatggacggacggacagatagataggtagaaatgtaaattacagggctacgctcagtggctcatgcctgtaatctcagcactttgggaggcgaaggcgggcggatcaccagaggtcagcagtttgagaccagcctggccaacatggcaaaaccccatctctactaaaaatacaaaaattagccaagcatgctggcatgtgcctgcaatcccagctactttggaggctgaggcaggagaatcacttgaacccaggaggcggaggttacaatgagccaagatcatgccactgcactccagcctgggccacagagtgagactccgtatcagtactttctttttattgtttttctgttattatagtttaagttcattgttattagattatatactctgtatggcttcaattcttttaaatttgttgaggtttgtttaatggtcaaagacatggtctgtctaggtgaatgttccatgggcttttagggaaaaaagtatattctagtgttgttgaatggtgtcttagtccattcaagctgctataacaaaataccgtaaactgggtgatttataaacaacagaaatttttctctcacagttctggaggctgggaagttcaagatcaaagtgccagcagattcagtgtcatgtgaggacgtgcttcctgcttcatagataagaggtacatacacgtttaggagcatcgtgtcttcctggtggatgaattctgttatcattaggtgatcctttgagcacttttaaaaagaatctgttggccgggcgcagtggctcacgcctgtaatcccaggactttggggggccaaggcgggcagatcacgaggttaggagattgagaccatcctggctaacacagtgaaaccctgtctctactacaaatacaaaaaaattagccgggcatggtggcaggcgcctgtagtcccagctactcaggaggctgaggcaggagaatggcgtgaacacaggaggcagagcttgcagtgagccaagatcacgccactgcactccagcctgggcaacaaagtgagaccctgtctcaaaaaataaaataaaataaaataaaaataatctgtttaatagcctactagtgttcttcctttactattttattgagcattaattaatcccaacattatgtctatgtcaggactgatgacaatatttggtataaaaatttgatagtctcagaggctgaggcaggagaatgcttgaatccaggaggcagaggttgcagtgagctgagaccgtgccactgcactccagcctgggcaacagaacaagactccatctcaaaaaaaaaaaaaaaaaaatcgatagtatcatatcctccaggattcaaagtgaacttcaaacagtcttatgtagtctaaattttggaatgcatcccagtattgagttgcagcagggatttgagtttttgtgaagagagagaggtatatcagaatcttgggcataaactaaggagccatgtcagaacctcaggtgtatgccaatgagatagatcagaacctcaggcatgtacccgatgagacagatcagaacctcaggcgtgtacccggtgagacaggtcagaacctcaagcgtgtacctgttgagacaggtcagaacctcaggcgtgtagccagtgagacaggtcagaacctcaggtgtgtacccagtgagacagatgagaacctcaggtgtgtaaccagtgagatatatcagaatcttgggtatttacccaaagaggtatagcagagtctcaggtatatactcaagaaggcatatcttgaggctttaagtatctagctaaggatttatatcaggatctcaggtttatacccagggaggtatagcagaatttggggtatagatctaaggaggtctatcagtctagagcatatagccaaggaactatatcagaacctcaggcacctacccaaagaggcattttaggactcgtaaggagggggtagatttcaaaagtgtagtctaacagtttatctactttgaaatttaaaacaatattaaaggaaaacatgaaatatttctatctgtcagaaggtgacatgagttttaaacaattaagaaatatactggctgtggccttgtaaccaaattattatgcctatagaaattacagactccattttccaggatagaataacagggactgacttaccttctcatctgagataacaaaacctccatacaaatacatgaaacaatgttcttcaagatgctggacatcaggcagtgaagggcactgatggttgtaagacaaggtgagaggtgtggcttgagagagtttccaggttgcagtgcagggagaggggaaactgaggcagatcttggcagacttcctcagttgacaaaatagagctgagagtccagggagaccatggtgtatagattatccaaagcaaagtatgagaggtgcaagccatatacagagggactccagagatctaccaaagtacttcttggtgcatccatatgagcaaaactacttgaggccaggaaaagaaccatctgagaggattagaaggaacagtgcccagtacttgtgccagccaggaatggtgcctgatactcacgcagggccaggaacagtgcagggatgtgagtgtttgttaggagagggaggtatatcagaatcttgggcataaagacaagaaaccatatcagaacatcaggtgtgtaccaatgagatagatcagaatctcgggtgtatacacagtgagatagatcagaatctcagatgtgtacacagtgaagcagatcagaatctcagatgtatacacagtgagatagattggaatctcaggtatgtacccagtgagtccaagagcatggtgctggcatccggtgagggccttcctgctggatcgtgacatgaagcaaggcaaagagcctgtcagctcagggctctcttcctcttcttataaagtcaccagtcctatcatgggggccccaccctgatgatcttataatcctaattacctcccaaaggctaccttcaaatgctatcaacatatgaatttggaaactaagtttccagcacatgaaatttgggggatacattcaaagtatagcaaatattacatcataaccagtaggattcatcccaggaaatgccaaatggcttgataatcaaaaattaatgtaactcatcgtattaacaggatgaaaaagaaaaaccatgtgatcatcttagtagatgcagaaaagcagttgattaaatcccacattcatttctaacttaaaaaaacaactggattttgacagaggtgcaaaggcaatttggtagagaaaggacagtcttttcaataaatggtgctggtgcaatggttatccatatgcccaaaatgaactttgacccatgcctcatgccatacacaaaaattaactcaaaatagatcagagatctgaaggtaaaatttaaaactataaaacttctagaagaaaacacaggagaaaaatctttgtgaccttggtctaggcaaagatttcatagatatgacaccgagaacacaatctatgaaagaaaaaaatcaataaattgaacttcatcaaaatgaaacttttactgttcaaaagacagttttaggagaatgaaaacacaagttacacattgggaagaaatattcgaaaagcatttgcctgataaaggtattgtagctggaagacagaaaaaattctcaaaactcacctagaagaaaataacccagttttaaaaatgggcaagagatctgaacaaacacattgtcaaagaagatagatgaatagcaagtaagcatgtgaaaaattctcaatgttatcagtcatcagagcaatgcagatgaaacctacagtccccatgctaatgttctacaacttacacagtggtggtatgataccactacatgcccatttgaatggccaaaattagaaaggttgaccataccaaacattagccatgatgtgcaggaactagaactctcatctttgctgacaggaaggtaaaatgatacaaacacattgaaaaacaggttggcagttgcttttttttttttttgagatggagtcttgctctcccaggctggagtacagtggcgcgatctcagctcactgcaacctctgcctcccaatgaattagaaaaataataataaaggtaacaatagcagtaataataatagaaataatgatagtttctttaataaaaatgctgtttaggcccagactgaaaggctttaagtaaccactcccccactgaagttagagttaagaaagaatattaattttccttgtgtgaaacattaatcttatctagcctccatgtattttgtaagttctgtaaattcctgttttccctgcacagctgcaagttcacaaggcagataagcttaagctgcaaaacatgtttttcttaagatgtaaggcatgtcacaagaatatcacaagatgataacggcctttattctcacttctgtatgcctgcttcctgcctcacatatttcctgcctcaagatgcgtaaaaggtacttgccttctttgtttggtgctctgactttctggatgcaagtccactgagccagtgtacaccttaaataaatcctcctgaaccccatcaatcgctccagttctctgatttcccactacattttctgggggctcgtccgggattggagatggcagattttctgtctcccttgcctgtggaactggagcccgggtcgagggagacctgggacctttggtgccaatgggaggactttagcccggaaaggagattggctctcctgcatcccggtgtccttcctagacagcacaacggaacctataaaggggttgcaggacggttccagcaggggctggggatggtgagagtagctcactgattcagatgacagggttttgccatgttgcccagacccagaggggctggggacagtgagagtagctcactgattcagatgaaacttacaccttagccgatgcaggacacgagagtggctcactaagttggtcaggaaagaaactgaaaatgggaagagtggcttcctgccttgactaaggatcgggaactgggagcggggaggtgtgtgaaagagatggttccgggagggccgtgatgtggggagacacagatctcttagcacggactgtgtgctctgaggcgagtgtgtgattgaccagaaccagggcatcacatacagctgacaggagctgccccacagctgcagcaggctgtggcaggaataaggtactctcctagctaagcagcacctgaaacttccgtaataggacccagtctggtcagtctggaacgaaagtgagagtgagtgtgcatcacaaagggcgggatgggaggaaaagcatcgaaacccactcctctggggtgcatgttaaagaattttaagaaaggttttgctggagattatggaattaagttgtcccccccaaagattgagggttctgtgtgaagtggaatggccttcttttaatgtcgggtggccagccgagggtacaataaatagggaaatgattggtcatatatttagggtagtgactggggttggaggacaccctgggcatccagatcagttcccatacatcaattcctggatgatcacagtctagacatgccccaaatggttacagccttgtctggcaacttactgtaagactctagtgacctgagccgaacctaaggcagttagagggcccccttcaccagacacctcaggtggaaagaaaaagccacaggaaaattaggaaagacctgttctacttcactgggatcaagtgattctcctgcctcagcctcctgagtagctgggagtacgggtgtgcaccaccacgcctggctaatttttttaaattttatttttagtagagacggggttttgccacattggccaggctggtcttgaactcctgacctcagacagtctgcctgccttggcctcccaaagtgctgggattacaggtgtgaaccaccatgcccagccagcagtttcttataaagttaaaccaatgcctaccatgagatctggcaatcccactcctaagtatttggccaagaaaaaagaaagcatatattccatacagagtctagtcctgaatgtctatagctgctttatttataatagctcagacttggaaaccattcagatgccattaataggtgaatatattctcaaactgtggttatccatacaatggagtattactttgcaatcaaaaggaatggcctatgaatacccataacaacatggatgaatgctgaaataattgtgctgagtaaaagaagacaggaaaaataagtataatacatactgcttgattctatttgtataaaactagaaagtacaaactaatctgtaatgacaggaagcagaccagtgacagtgggcatggaggggcaagagggagagattagatgggcacaggagagctttgaggatgatgggtctgcgtactgtctcggctatgatagtggtttcacaggttgatacatacggcaaaaaataccaaatttgtacactttaaatatgtacagattattgtatgccagttacatgtccataaagctttcttttgttgttttgtttttattttattttttgagacagagtctcgctccatcgtccaggctggagtgcaatggcaccgtctcagagcactgtaacctccgcctcccgggttcaagcgattctcatgcctcagcctcccaagtagctgagactacaggcatacgccaccatgcccagctaatttttctatttttagtaaagacagggtttcgccatgattgccaggctggtcttgaactcctgacctcaggtgatccacccacctcggcctcccaaagtgttgggattataggcatgagccacagcaccgggcccataaagctgtcttttaaatgaaaaaaagttgtcttgaaataagcattagaactgtggctttggctctgaaatcctcatctgaggacccacactcgggtgccccaatgtggcggtgcttacagaaatgactccatctgctaaatgagtaaatgggtaattctccactgaacacacactcgtttagcagcataagcagcaagagttcaggtaatcctcacattgcaatttgtcattagtttaaacttccagtctttgttttaaaaacacattagaataatactacattttccctcatctctaaacttgactgaagactccaagagagagtaatattcatcaagaggatcatctactcaacacagataaactgggaaagaaaaataacttgtgagtaattcagaatctggattatcaggtcaggctcaatggctcacgccagtagtcccagcactttgcggggcccaggagggcagatcacttgagttcaggagtttgagaccagcctgggcaacatggcgaaaccctgtctatacaaaaaatagaaaaattagccaggcatggtggcatgtgcctgtagtcccagttacccgggaggctgaggtgggaggatcacttgagcctgggaggtcgatattgcagtgagctgtaattgcaccatgcactccagcctgggtgaaagaaggaaactctgtgtccaaaacaaaacaaaacaaaacaaaaaaagctaaattatcaaatgtctagatcgttgatggttggaagtaaagttgagaaatgttcacactgggagatgacacacagtaaaccacacagagggttctaacgtggttgttagaagcagaaactagaggcttgctgcctgaggtcaaaccccggtcccggtggttctgtgccccagcgcatgttgtggtagcctctctgtacttcagtttcctcatctgtaaagtaaacataatgataatgcctgcctcatggggttgctgttaccaggaagtgagttaatgcacattaggttcttatttatgacagtgcctggcataggataagggctcaaaaagtgttagctggaactactatcattatcaacatctctaatttattgcagggttggatctgaaaaatggctgatgatgatttgatgatgacttcatttttataaaacaataatattgcagtgcaaattaaacacaagcaacctgcaacacgccactgcaagttggatgtctagaaaaggtgccatgagttaccttctaaaacatcataagaaaccatgttcaccaataattaccataataggagagaagtaccaagtaccatggggagacagagtccagaatctcagagagagacacagttaccttttagttacactaatggggaaaacaggagctttgctacccttgcacctgatggagggcttctctgaatatagggctatggggtcagaagccagtttcctcccatatttagaaggtttccaactgttatctttcacttcccatgttgctgttggaaaatccaaaagtattctatttggccaggcacagtggctcacacctgtaatcccagcaatttgggaggccgagattacctgaggtcggaagttcaagaccagcctggccaatatggcaaaacctcttctctacaaaaaatacaaaaattagccaggcgtggtggcgcacgcctgtagtaccagctattcgggaggctgaggcacgagaattgctttaacctgggaggtggaggttgcagtgagctgagattgtgtcactgcactccagcctacgcgacagagcaagactccgtctcaaaaaacaaaaaaagtattctgttggatcgtttgtgtgcgacgtgtttttccctctcagaaagctcgtagggtcttctctttgtctccagcatggtctggaatttcccagtgagtgaccatctgtgtgtgtgtattcatccattccatggagtccctgctgggcccttgcaatctggaaattcatgcccatcatttctgagaagttatcctgaacgtactggttggtggtttcctgtgctccatgttcttgcttcctgctcttcggagctcctgttatttggttgagttttgtctcctggactggtcctctcttacttctcttgcttctcccatgttccatctgttttcactctactttctgtgagatcaggccctttatcttccaacccttctattaggtttgcaattgagtttgtaattccctagaaaagttcttattctctgaatatcccttttgatagcatactcttcctttttcatgagtgcagtgtttctgcatggctctcatcagaacatgctagtgtctcccatttctcataactttctagagtgaggaccatttgaacttggagtgccctcattttaaaactctgtggttgaccttgttcccctcttttgctgctgcttttcaccagactttgaagaagcagaagtacattcagaacttgtctgctctggcaaaagacaatactgttggcttaatctaaaaattgaagaagaaagctcaaggagagaagtttaaaaatataccacctctggctgggcgcggtggctcacatctgtaattccagcactttgggaggctgaggcaggtggatcacctgaggtcaggagttcaagaccagcctggccaacatggtgaaaccccgtctctactaaaaatacaaaaattagccaggtatggtggcagccgcctgtaattccagctactcgggaggctgaggcaggagaatcacttgaacccaggaggcagaggttgtggtgagccaagatcacgccactacactacagcctgggtgacaaagtgagactccgtctccaaaaaaaaaaaaaaaaaaaaaatatatatatatatatatatatatatatatatatatatatatatatatacacacacactaaccttcagcatataggactattgcagaagggattatctttctacttggttggttcctcttggtcttgagcaaattttgacttccctgagttggcccctaaaagttaaagggaaagggccttttctctttcctttaaaaccaatatggcatatttgctgagaacttagataccacaggattggcagtgtagacttacattcatagaccggatgccatcagccaaccttgagtaatttgcagcacactgcatcattttatttaagtaatgcgaagtccttgacatgtctcagacattgtcttggttacttgtaaggtctcacataaatctaattttcctctttctctgccctttctggttcagctcagtttattcaagggtgtatttgtgcaacacacttgaataaggtgtggtcccgcctttgtagatgttatagtttgggaagaccagccgggcagagagaagagcatgattcaaggatgaaggcgtgggctgggggccgagggagcaaggattcccagtaacgagggaggaaggagcagcaccatgtgcccattactctatagacatctcgaaccacctggccatgtagctgtcattaacctaaatttacagttattgaaactgaggttcagccaggcgtagtggctcacgcctgaacacaggaggcggaggttgcagtgagccgagatcacgccactgcactccaggctaggtgagagagcgagactctgtctcaaaaaaaataaataaataaaagaaaagaacaaaactgaggttcaaagaaatgtacagtgctcccccccttatccaaagaggatacactccaagcccccacagtggatacctgaagcctcagatagtatcaagccctatatatgctatgttttttccctgtatatgcatacctatgataaagtttataaattaggcacagtaggagactaacaacaatgataataaaatggaacaattataacatacactgtaacaaaagggtctcttcctctctctctcagaatatcttattgtactgtactgggggtaactaaaaccaaggaaagtgaaaccatggataagggatatctactgtataaggtggagttttcaaggtcatagcactgccttcccctgaggttggccttgcagcctctctaggcactgctgctgctgctaagaacccctgtgaggtgaacactgtaagcatcatcattgcttctcagaagaggagacctggcttacagaggtcaagcctcaggtaccttaaacaccattttaaaactgaactcatggccaggtgcattggctcatgcctgtaatcccttctctccatgctcaaaacctgccctccttgtctttatattccaaatttcgtgggtgccacctcctctgcccagtgacttaagccagagcatacattcatcctagactctgtcccaggtccctggtccaggcagctgccagttgtcaggatcagctctttatctcgcagtcctcctgcctcttgtgtcattacccagggctgtcaccatcttttcttgggacagttacaacagccccgtaaggagttgtgctgcttctagtcttgttccctttgaatctggattccttcttgccatcaagacaatcctgatacaaatctgatcacgtcacacttcccttcaatagtcttccatggctccttattgttttaggatgaaatccaaactcctaaacatggggattaacaatgtgccatgattggcactgctggcctctcctacctctgcagactcacctcttgccacttctcccttgaggtagatcaaaaatggtcacaagttctttgaggctcttcccatcaagaggtagagtttatttccccacctcttggatctggcttgccttgtgacttgctttgacccacagaacgtaacagaaaggacactgcctaacttacaaatgaggtctaccttaagaggctttgcagattccacattcaacctcttggaatgctgccaccatctgagaagcctgaggtggcctctgtgaggatgaaagacttcatggtgagaaatacctagcgaacagcctggcaccagctaccaggcatgtgactgaggccatccagccatagctgagccacaaaatgaccacagctatgtgaattatcccaggtcagaccagtagaagagccacctggctgagctcagcccaatttgctgacccatagaattgtgaacaaataaaatggttgtagttataagccattaagtttcagagtttgttacacggtaacatgtaactgatacaactcttggagccagttgttcagccattctcaaccacttattcaatgatgttttgggccatatatgcagatatgctgttcccttttccttgaaatggcccttaccctcctttctgttgggttttcctatggaatatccagtcagcctttaggattcatcttgggtgtcccttcctgtatgtaggctccctggccctccaggattcccccagtaacagccctcatcatgctgcctttgcaaccatttgtttatttgtacctctcacctgctagttgggcaagttactcacttctctcaacctctgcatttttcttctttataaatgggaccaataatacctaccctgccctggcgtggatagattaaagaaaaaaaatacatgcagctgccattgagggcctggcccacgtgtgatgttcaataatattatttctccttgttttccttcccgtgccagtgccacacccccctgtcccagtgcactggggctgtggatcccttcaaagctgagattgcctgtctgtggtctccagcgttaagcacagtcattagctcaggtgcgtactcatgtgttccacgagttcaagcctcagccctgtaaagtttgcctgccgtgtatctgatatatttctgctaaaacccattaggcctttcttgctctgaaatgtcatcgttagttgtgtgtcacttcagttttgtaactggccaggccactgcgcccaggctgcttcctcgtcatctggctgctaaatgcttcaaccttacctgccttgctatgcgtcccatcctgtatcaggtcagagctcttgagtggtgaatacaaatttcatttcagttgacttttgattcttgtggcaggcctctcggcctactctaatttgattgcaacggacacaaaatgtgtccaaacttgcagcttttcttctcttattttgatatcaccatccacaaaggtaagatattttaaagcaataactacaaactttctgaaaattatgaagaagtgctgggttttaaatggaagtcatatagtgtgaactttgtgtaaagtccgtagggagttttcttggaaatggctgggaacattctttttgcacctttgaagataaaggtaggtggaggagctcacagctcttgtgccatgttgggcttgtcactcttgtttatgtgccaaattcttttgattacaaaattttaagtttaatgctttaggtattgttgggcaagatctagatgtatctagttaaatgtaggtgatatgcaaactatttatgatgtatttgatttaaattcattaagatagagtgtctttaccaccattatagtctggtccttttccttctgttttaaatgtgtttccattggcattttctaaactgactttgttagcgtgttaatcatttggcactggtaatgattaatcttttctttctttctattttttttcttttttttttttgagacagagtcttgctctgtcaccaggctggagtgcagtggcgcagtctcagctcactgcaacctccgcctcccaggttcaagtgattctcctgcctcagcctcccaagtagctagggactacaggcacgtgccaccacgcccagctaatttttgtatttttaatagagatggggtttcaccatgttggccaggatggtctcagcctcttgacctcgtgatccgcccacctcggcctcccaaagtgctgggattacaggcatgagcgactgcgcccagccgtgttcatctatttctgtgaaccgatgctaggtgaaggtacagagggctttctagcttctgggtttgtttattctgaaatgttattttaaatcttagcccaacaaattgagcgaaaagacttctagatgttaaatatgatattcaaaaaatataaagacaaggtgataaattagaattggtgggaaagagaaaaatctgtcttctgatggtcacctgccccagcaacactactcgtttgagaagacttccatcctttaccctcaaagtgttccatgaggttggatcagacatcatttagcaaagaaagatgtaaatagatttctgtagggtggcattattaagcatattaagtggttacaatacagtaaattagagggagtagtacagaagcataagcagtcaaaaaagtgaaagtctaacgttcgtaattattgttctggaggcttttgtatcacatataagttccaggctgggtatgatggctcacaccagtaatcccaacacttagaggccaagccgcgtggatcgcttgagcccaggagttcgagaccaggctgggcaacatagtgaaacctatctctacaaaaatacaaaaattagctgggggtggtggcagcgcctgtagtccaaaccacttgggagcctgaggtgagaggatcacctgggcccgggagatcaaggctgcggtgagccatgatcttgccattgcactccagcctgagtgacagagagagactctgtctcaaaaataaaaaagttttgagtgtgaaaattcaagctcaattccatttgttggttgtcttgagtgtctgatcacatagaatataaagatgttttgatagttgggacagtattcagctacctgctatttaatacattatttcagaaaatatttacaaagggggctgggcacagtggctcatgcctgtaatcccagcactttgggaggccgaggtgggcggattacctgaggtcaggtgttcaaaaccagcctggccaaacatggtgaaaccacatctctactaaatatacaaaaaattagccgggcgtggtggtgtgtgcctgtagtcccagctactcaggaggctgaggcacgagaatcgcttgaacccgggaggcgtggggttgcagtgagccgagattgcacaactgcactccagcctgggtgacagagtgagactgcatctataaaaacaacaacaaaaaagaaaatatttgcaaaggaccttctgggtccaagaacctcatgtccaatacaagggtgcacacgtgggtgagacacggcagctgctctccagaagcccacagtggaggggtttcccttcggtctccttttattccaagcaagtggcaaaactactttactcttaatacaaaccacttccttttatcacaggacgcttcccaagctctgcaactgttgctcctgaggaagggagtggaactgataatctgttcctccctattgtgttcagtatggttttttttttttttttccttttgctggctttgttttcctgtccctgtgatgattaaaattcactctgcaaattagatcacctttcccacgcagagtccctttgacttctgttctagatatccattacatttttgtagtcttcggacacactgtgtgtgccgctttgccctctgggtgacagcaggctgtggctgcggcgacagagctgaggtgaattctcacagaccatcactgggttactcctggagtaagtaattcccaagagctccttctgtgcagatcgttagaaatagatattgaggccaggcgcggtggctcatgcctgtaatcccagcactttgggaggctgaggcgggcagatcacgaggtcaagagatcaagaccatcctggccaacatggtgaaaccttgtctctactaaaaatacaaaagtagccgggcgtggtggcgcacgcccgtagtcccagctactcaggaggctgaggcaggagaatcacttgaacccgtgaaacggaagttgcggtgagccgagatcacgccactgtactccagcctggtgacagagtgagactccatctcaaaaaaaagagaaagaaagaaatagacattgaacacctgctacacagcagggattgtgctagaagtatggatgcaaagattaggtgaatatgttccctagcctcacaaagcatacagtctagtaggagagacagacacgtaaaaagtttcaacagcacagataatcagggctacaccagaattgggcccaagatgctgcaggaatctataggtgaatgggtttcatgaaggaagagcttcttctcccatttataactcattttagcctaatcttccaaacagtcacgcatctaagagcaggtgatgcagaaaataccctcgtgttagttatgaattaccgttggaatccttccagtgtttgcacctgccctgtgctcgggtaacataaaacagtgatataatttgatgtctacttcctcttgtatttgtctgtttttaagtgttctacaattttcatatactctgtttcatcgttctcaaaggaatattttgattgataaatgtttagttagtaagacctaaaaactgaatctcagtagtttgagcttatgatatacaagatgcagctctaacatttaaattggaagggaaatgtcaaaaagatacctgcactcttgtttgttgcaacactgtttacaatagctaagatttggaagcaacctaagtgtccatcaccagacaaatagataaaggaaatgtgatatatatacacaatggagtactattcagccataaaaaagaatgagatcctgtcatttacaacaacatgggtggaactggagatcattatgttaagtgaaataatccaggcacagaaagacaaacttcacatgttctcacttatttgtgggctctaaaaatcaaatcacttgaactcagagagattagaaggatggttaccagaggctgggaagggtggtgaggggttgggggcagtgaagatggttaacaggtacaaaaaactagaaagaatgaataagacccactaggttttttgttgttttgttgttgttgttgttttgagacagagtctcactctgtcacccaggctggagtgcagtggcatgatctcggctcactgcaacctccacctcctgggttcaagcgatcctcctgcctcagcctcccaaatagctgggattatgggcacgcgccaccacacctggctaatgtttgtatttttagtagggaccgggtttcaccaggttgaacaggctggtctcaaactcctgacctcaagtgatccactcgccttggcctcccaaatgctcagattacaggcgtgagccaccgcacctggccactgtttgatagcataatagggcgactatagtcaataataacttaatggtatatttttaaataacttaaagagtataattggattgttgtaactgaaaggatcaatgcttgagggcacagctaccccattccccatgacgtgtttagttcacattacatgcctatgtcaaagcatctcatgtaccccataaatatatacactgagtatataccacaaatattttaaataatttttaaaataaaaaaataaattgtaagggaaagaaaattatgaatttagaaatgtaaaaggtctcaggtaaggaaggaatgagaggatcatgcagaacctcccatcattgctgggactggaacagaagccctaccttttcccaacaccctatccacctgtccctcacctctcagcttttgtgagactctgtctgtgctatgaaactgaagatctaattcagtgctgtttgcattgtcttgcctcctggaccagaggttgcagttgttgagaaaagggatggttggttatgccttgatcccccccagagcatttggggcataggacacgggaactggccagcctggttcactcttctcgattagctggacagcggcatgtcatgtgggtaataggaaggggtggggacttccccgggatattctgctcctgatcagaagcgccagtgatgtggggggagccccagcaccagagcatgctgggagggcgtgcagggtggggcaggtgcccgtttggcctctgctgtctatctgggggatgcatccaaaggcaactgttccttatctgctcttgttgggagcaaggaagggccaatttgttcaatgatccgtatacagccagtccctctggccagagttcaagacagtattgcctcactctatatagagattgtatcttggttagctcttcattcatagcaagaccaatgtttctgtaaattaatcctggtattgtttaaaagcaactaaaaatgatgaaattgtaaaactttgaaactccctgaatataacgacaagcaaactaacattgttttattggtcgatgctcctggccagaagagagaatattagcagggataaaaggcataggccacatgcattttccaccccagtgctgagaacacgatgggcgaaaaagggaggtggccacagcccatccatcacacagtctctgcccatctacttgctttttcctttttttttttttttttttttgtgacagagtctcgctttgtcacccagactggagggcagtggtgcaatctcagctcattgcaacttctacctcccaggttcaagcgattctcctgcctcagcctcccgagtagctgggattacaggcacctgccaccaagcccagctaatttgtttgtatttttagtagagacggggtttcaccatgttggccaggctggttttgaactcctgaccttaagtgatcagcccacctcagcctcccaaagtgctgggattacaggtgcgagccaccacgcctggccccagctacctgttttctttcttttttttttttttttttctttttttgagacaaagtcttgctcttgtcccccaggctggagtgcaattgcatgatctcagctcactgcaacctccacctcctgggttcaagcgattctcttgcctcagtctcctgagtagctgggattacaggcgcctaccaccacgcccggctaatttttgtatttttagtagagacggggtttcaccctgttggccaggctggtttcgaactcctgaccttaagtgatctgcccgcctcagcctcccaaagtgctgggattacaggtgtgagccaccatgcccggccccagctacttgctttctattgggatgaacctcatggttaatacagttagttagtgactgcaacttttgaactttttgttcatagtgaaaaatattttaagtaatgcttaccccattatgtttcttgtcatttgaaaaaaaatctcccttcagacagaatgcagaataaaatactacagaaaatctgtacagagtcccagcctgacttatgctagtaggttacagagaaagaaagtcttctaaaccctatgaaaggttaacagttctcttatttttccctgtgtgctatttgatgatttccctgtgaactttgatgatttattgccagaattccaaacataatatgtgaatttcacaaaaatggatgaaatgtatctatttttcattggtagaagaagccaaaacatcccttcctcaccgcactaaaagctgttgtttacatgaagcaaacctcaaatgtgaacatatttttacgcaaatgcatttaatgggtgaatatttgctttgggacggtattctttactctatctggagagtctggcgttccgtaatcaccatgtgatgacggctgccctgacagtggctggtagcagcacatacccccgagcctctccgtggtgtgcgccgtgggcaccatgtgaccattttcagaaaggaagacagttctggaagctaaaggtcacctagtcagcctcgttgggtgattgatgactcagctgggttcagggaggtggacccgaggcagagcctctagaaggcagcggtgggcagggcggttcaggcaggtggcacctgggcaaaggtgcagacgtggaatcctgaaagcaattctcagcgctgctgcgtttccaggaggtagaagaacagtgacaagtgcacagtcgggtagggacaaatgtggaagggctgggaacagtgtgttcaggagactgggcttcaatctggaggtctcaggaagtggtttaggatgtttcagcgagagcatgatacagactaacccaggaagaaccgctgctttgtcacttatacccctatggaaatgccgttcgctttgctagttgaaatagcctaccattgtctgggactcacccagttagatttgtttggactccacaaagtattcttgaccatacaatcatggtcgaggaccccctacatgagctgccttcatggctacagggagagcacaccaaagtggatgtcacacccagcacacatgccaccggcttggccctgcgccccgcagcctgagccacactggctgcctgttcctggaatgtgccaacatgtttcagtcctggagcctttgcacttggtgttctcttcgctggaacattctcccccaagacatttacacagcttgccccctcattccctgaggttatctcctgccccctaatcagtgaggccttccctggcctcaccccggacactccacacgtgcattcatttcgttgttcaccatctgtgtcccagttacaagggaggctccctgagagcagggatctgatttttgttagttgttgttgttgctgttttgaggtggagtcttgctttgtcgcccaggctggtgtgcagtggtgcgacctcagctcaccgcaacctccgcctcccatgttcaagcggttctcctgcctcaacctcctgagtagctgggattacaggtgcctgccaccatgcccagctaatttttgtatttttagtagagacagagtttcatcatgttggtcaagctgccctccaactcctgacctcgtgatctgcccacctgggcctcccaaagtgctgggattacaggcatgagccactgcacccgaccctgttttttgtttggttttggttttggtttggttttggtttttttttgagacacggtctcactctgtcgccccggctagagtgtggtggcaccatctcggctcactgcaacctccacctcccaggttcaagtgattctcctgcctcagcctcctgagtagctgggattacaggcacatgccaccacacccagctaatttttgtatttttagtagagatggggttttgccatgttggccagtctggtctcaaactcctgacctcaagtgatccgcccgcctcggcctcccaaagtgctgggattacaggtgtgagccactgtgcccggcccagggatctgtttttgtctccgctgtgtccccagcacctcaaacatattgtacggagctgcgacagctgcgcagtcagtgatgactgagagattcctggccccgtgggctatggctccttcaacagtttgttgtttaaaggttcttcactttctcagcgtgctgatcaagagacaagcctggaggagaggctcagtggtgctcctgtgtagatgatgaattcaggtgtatcttggatggtaaatgacgttgcatttaaaaccaagcaagtggccaggcgcagtggctcacacctgtgatcaaagcactttagaaggccgaggcgggcggatcacctgaagtcaggagtttgagaccagcctggccagcatggtaaaaacccgtctctactaataatacaaaaaaactagctgggcgtggtggcgggcacctgtaatcccaaccactcagaaggctgaggcaggagaattgcttgaacccgggaggtggaggttgcagtgagctgagatcgcaccactgtactccagcctgggcgacaagagcaagactctatctcaaaaataaaaaaaattaaaaattaaaatttaaaattaaaacaaacagccggacgcagtggctcactcctgtaatcgcagcactttgcgaggctgaggcgagcggaatacgagctcaggagatcgagaccaccctggctaacacagtgaaacccgtctctactaaaaaaaaaaaaatacaaaaaattagccaggcgtggtggcaggcgcctgtagtcccagctactcaggagactgaggcaggagaatggtgtgaacccgggaggcggagcttgcagtgagccgagattgtgcccctgcactccagcctgggcaacagactgagactctgtctcaaaaaaaaaaaaaaaagaataaataaataaataataaaaaataaaaacaaacaagtgaacgttgttatacgtcagtcttaccaattgttcctctttcctcccagtagcttggagctcggcggcacaaccagcaccatctggtcgcgatggtggacacggaaagcccactctgccccctctccccactcgaggccggcgatctagagagcccgttatctgaagagttcctgcaagaaatgggaaacatccaagagatttcgcaatccatcggcgaggatagttctggaagctttggctttacggaataccagtatttaggaagctgtcctggctcagatggctcggtcatcacgggtaagtgtgccgtttcctagaaagttttatttagaaatgtttcttcctccaagaaaactgttctctcttttttttttttttttttttgagacggagtctcgctctgtcgcccaggctggagtgcaatggctcgatctcggctcactgcaggctccacctcctgggttcacaccattctcctgcctcagcctcccgagtagctgggactacaggtgcccgccaccacgcccagctaatttttgtatttttaatagagacggggtttcactgtgttagccaggatggtctccatctcctgacctcatgatctgcccgcctcggcctcctaaagtgctgggattataggcgtgagccaccgcgcccggccgaaaactgttctctttagctggaaaagaagtcacacttttttgcaaagaaagcttcagacgtggtaaagcatgacctccagtgcccctgggccctggaaggcgcgtgtcacggctcacggtgccccctcttgtgaaagccatgcacacatcaaacagtgcttgagattcagtcacggggaacagctaaagtacacagaccctaaccccagcaagcccgcggggggcagctagacatttttaagaggagacgtgtgcaagggtctgcatagaggtactgttggtaagagggaaggatgggaaacaagctgtacatgcgtcaaagggaaacagataaattgggatgcatttatacagtggtatatacttcatagcaatttaaaagaacagactaggctaggcgcggtggctcacgcctataatcccagcactttggaaggccgaggcaagtggatcacttgaggtcaggagcttgagaccagcctgaccaacatggtgaggccccatctatacaaaaaaaatttaaaattaaaaaaaattagccaggcatggtggtgcatgcatgtggtcctagctactcaggatgctgagggaggaggaccacttgagcccaggagctcgaggctgccatgagctatgactgccactgcactccagcctgggtgacagtgagaccctgtctttaaaaaaaaatttttttaagcaacattgaatgaaaataaacaagcttaatgaatatttttatgatccaattaatgtaaaatcttttattttttattttttgagacagagttttgctcttgttgcccaggctggagtgcagtggtatgatctcagcccactacaacgtccatcttccgagctcaagcagttctcctgcctcagcctccctagtagctaggattacaggcacccgtcaccatgccgggctaatttttgtatttttagtagagatggggtttcaccgtgttggccaggctggtctcaaactcctgacgtcaggtggtccgcctgcctcagcctcccaaagtgcagggatcacaggcatgagccactgcacccggcccaattaaaatctttaacactaaacaatctagtacatcactggtggaaacagacatacacctattgcaaagggcatctcagctttaaggactcagtcacctcctgagcaagatggagggagaactggggaggggtcccatggggactgtaattctctctaggttgtatatttttaaaagacttcagcagtgtgataaacctgggtggtgtgtacatgggtattacagtcatgttgcttaatgacagggacaggttgtgagaaatgcatccttaggtgatttcatcattgtgtgaaagtcatagagtacacttaaacccagatggtagagcctgctgcacaccgaggctctgcggtgcagcctgttgctccaaggcacgcacctgtacagcgtgttactgtactgaacggcgtaggcccctgtgacacaatggtaagtatttgtgcgtctaaacataccaaaacatatagtagaaaaggttacagcaaaaatacagtattatcatcttatgggaccatgataccacagttgaacttatggtctattgttgaccaaaatgtcactgtgcagtgtgtgactatacagaaataagctcagagaaattaagtaacttggctgggcgcagtggctcacgcctgtaatcccaacactttgggaggctgaggcaggcggatcacccgaggtcaggagttcaagaccagtctggccaacatggcaaaaccccatctctactaaagaatacaaaacattagctgggagtggtggcaggtgcctgtaatcccagctactctactcaggaggctgaggcagggagaattgcttgaacccaggaggcagaggttgcagtgagcagagatcatgccactgtactctagcttgggcgacagggtgagactccatctcaaaaaaaagttggggcgtggtggctcatgcctgtaatcccagcactttgggaggctgaggcgggcggatcacttgaggtcaggagttaaagaccagcctggtcaacatggtgaaaccccatctctactgaaaatacaaaaattagccaagcatggtggtacacacctgtaatgcctgggcaacagagcaagattccgtctcaaaaaaaaaaaaaaaaaaagtaagtaacctgccacggttcatacagccagaaagacacagagccgggcctggaccccgcctctcagcttgctctagagggctattctctgcatgctggcatgatcgcgccttgtaaaaggtggcagtgttctcagcttagtcaatcaggaattgcaagaggcaagtgagcccctgaggactctggggggcctttgtgaccgagcagctttgggagtgaccctgacagacctttacaggtggtgcaagttttgactccctttctcctggcgcgttaagcagaggataagcgctgtggaaggagtgaaggtgtagggagatcatggcccccagagcagtggggaaggggacagggaggctggaggagagcaaggaaaaggctccgtgtcaggtggcgccttgagtggcctgggtaggttgtcttgcagtgaacccgggttaatggccttgacaatgaccgcattgtttcctgagcactgcaggctgcccacacacctcacacctcggcttgcctaagcccagagcagccttgtgaggtcgttgttatgtttatttaaggaaggaggaaaggaggcaggtcccaggacatcctgacgtgctggagatcaccagcccagaacccagctcttaaccccacaatgtgggacctttcttcacccatcacagacacaccccatgctggttcaccgttttcctataatgactatttgtgctatttattagaaaaatcttttccttatggatttgaaaagatttatcttgcttttgtttttcttttttgcctttcttttttaaggcaggcaggctcccgcagccccacccccagggtgaaaaatatagttcattgtctagtaaaagagttcagagatacacttttttctttgggtaagatatactctagagcttgttctgaaatatggaatttgtgtgagctgcgggagtgggtgggtgtgtggctctagctctggaaagttctttcctggcagtggccaggagggctgcccagccccctcctgcctcctctggcagcttaaacacaggaccccttattctgtgctctctcctgacccctggtcctcatgcaggagggaaccctgctcttctagggtccttttctaaaagtagtgtcttttaggtcattgtcaagaactataatctaaaatgtatttttaactcatctggaaattctgacagaggtaaggcttgagaatttcctgcatactagccttgtggtctatataatccattaaaagccacatttaacccaattccacagactgaactgtgcttcccatctaaataaattaaaagcaggccgggcacggtggtcacgtgtgtaatcccagcactttgggaggtcgaggcgggtggatcacctgaggtcaggagttcgagaccaacctggccaacatggtggaacctcatctctactaaaaataaaaaaaattagctgggcgtggaggcgtgcacctcttaagcttaaggacatatttcttatgatccaattaatgtaaaatattttattttttatttattttttgagacagagtttcactcttgctgcccaggctggagtgcagtggtgcgatcttggcctgtaatcccggctactcaggaggctgaggcaggacagtcgcttgaatccaggaggcggaggttgcagtgagccaagatcacaccactgcactccagcctgggcaacagagtgagactctgtctttaaataaataaataaataaatagcgagggttcagggcaggagaaaaagggttccaaatttgttctgaaccaattccaaggaactttatggcacaaagaaaaaaaaggggaacttacaaaaagtgaccacactgaagcgtcctggtcacccatccctggttttgaccaccagcctttaaagtggcaagcgggtgataacccatttcttatttccccctcagcatttcctcactgttattcatacatgtggtcatttgtactcatctcacaattgttaaaacctctttcctcccttccaggttttactgaactgttactgcgaagtctgagagatgaggtcatttaagattatttcttatttgtaaattagatcgttcatatttgtacctaatctgatcttttgggtaatattcctagttatgtagactggtctctcagaagagccggatattaaatgcagtactttaaactttacacccaggagaccggatgggtgaggctggttcactcggccaaagtaccattttatctctgctttttcttcccggctttattgccataattgacatacaataaactgcatgtatttaaagtgtacaatctgttgggtgtacacacacacgcatctgtgaaaccatcatcacactcaaaatagtgatgtagaaattttgctccttagttcgactaaatctgggttcttgtgtcatgaccaggaaaaattaggcacgtggacacgttgaagggtgaggagagcagtattgggcgaaaaggaaaaaagaaaaaaactctcagcaaagctagaggggatcctgccaatgagttcccagctcacagactgattagcaggccaccacacatgagctggaggccaggctcctcccgctgcgcaaggtgagaacttcccgtggctccaccccattctcccaatgcccaggtgggtccccgtcccttgcgggcctgtccagacaagggaaccctgggcaggttccctcatctacacaaaagcacctgaggtaaacacttgtggggcaggttgcagattctctggggacgccccccttctctgcctcctgcatctatcagtagtgcctctgtctgtcacccctaaagtttacttgtgctgtttctaattcctctttccccagccccgtgcctccctgcctccctcccccagtaaaccatgaatccactttctatcattctaggttgctttatatttcctagaattttatataaatggaatcatacagcacgtactctttctaggctggcttctttcactctgcagaatggctgtgagactcatctgcattgcagcaagcatcaatagttcattcttcatccatcatgtggacatagcacagtttgctgattcacgcacctgttgatgagcatttaggttgtttctagcttatggctattacaaataaagctgctatgaacattcacgtacaagtctctgtacaaccctctgctttcatttcttttgaataaatacctaggagtatgacggctggaacagatggcaggtgtttgtgtaactttttaagaaactgccaaaatcttttccagcatttcagaaaaatcttagaaaatgctatactatgttatattcccactggcagtatatgggggagttccagttcctccataccctcatcaacatgaggcatgatcagtctttttaattttaaccatgtcagtaggtgtgtgatggtctctcactgtggtgatttttatttgcacttccctggtgattttgagcatcttttcgtatgcttatttgccatatatcttctttggtgatatttctgttcaaagcctttgctcattttttaattgagttgcttttctactattcactattgaacactatttatatattttgaatacaaatactttatcagacatgtgatctacaaatattttccccagtgtgtggtttgtctttcttttctttctactgatagtatcttaaaaaaaaaaaagaaaaaagattgttttgtttgttttgttttgtttttgagatagggtctcaatctattgcccaggctagagtgcagtggtgcgatcatggcttactgcagccttgacctcttgggctcaggaaaccctccgacctcagcctcccaagtagctgggaccacaggtgtgtaccaccatgcttggctaattttttttttttagatacagagactcgttatgttgccaggggtggtcttgaactcctggactcaagcgaccctcccacttcggcctcccaaagtgctgggattacaggtgtgagccatcatgcccgaccagttcttaattttgatgaagtccaatttatcaatgtcctttttttatggatacttcatttatttatttatttgagagagggtctcaccctgagcccaggctggagttcagtggcatgatctcagctcactgcagcctcaacctcccaggcccaggtaatcctcctacttcagcctcccaagtagctgagactacaggtacctgccaccatgcccgggtaagttttttgtatttatttgtagagacggggtttcgccatgttgcccaggttggtctcaaactcctgggctcaagtgatctgcccatctcagcctcccaaagtgttgggattacaggcgtgagccaccatgcccagccatatatatatatatatatatatatatatatatatattttttttttttttttttttttttttttttgagacagagtctcactctgttgcccaggctggagtgcagtggtgcaatcttagctcactgcaacctccttctctgaggttcaagtaattctcatgcctcagcctctttagtagctgggattacaggcatgtgctaccaggcccggctaattaccagccttatatttttgaactctgtttaaaacatttaggtgcataaacattcaggcttgttatattctgttgatgaactgaaccttttattattatgaaattgctgttgtaatccgtggtaaaattatttgttctgaacactactttgtctgttattgatgtagccactgcagctttcttttgattggtgttaacatggtatatcttttcccattctttttcttttaactggtttgtgtctttatactatggtttgatttaaatctattatctcacaatttgttctctttggtacatctttgttttgttcccttttcctctttttatgccttctgttgaattaattgagtcttttttgttttgtttcatttaattttgttttttgagacggagtctctctctgtctccaggctggagtgcaatggcgctatctcggctcactgcaacctctgcctcctgggttcaagcaattctcctgcctcatcctcctgagtagctaggatcagaggcatgcaccaccacgcccggctaatttgtgtgtgtgtgtgtgtgtgtatttttactagagacgggtttcactatgttggtcaggctggtctcaaactcgtgaccttgtgatctgcctgccttggcctcccaaaatgctgggattataggcgtgagccaccgcacccagcctaattgagtcatttttaagattccactttatctcctttgttggcttattatttataacaccttctggtgttattttagtagttgctttagggtttatagtgtatctctctaatgtctcccagtctaccttccagtggtatcattctatcttacagatattataagaactttatgacagtatactttcatttttcccttcatgcatttgtggtaatgtttcacataattttatttatttacctacattataaatattacaatatgttattgttttacatagacagccggttatctttttaagatagtagtaagaaaaattttttacatttacccacataattaccttttctagtgctatatacctttgtataaatccagatttccatctgctatcattttccttctgcctgaaagacttcctgtgatattatctataatatggctctactggtaacgaattactagcttttgtatgtctgaaaaagtcttcatataaccttcattctagaaagtatgtgattcaaagggccgggcacagtggttcacgcctgtaatccgagcactttgggaggccgaggcgggtggatcacctgaggtcaggagttcaagaccagcctgaccaataaggtgaaaccctgtctttactaaaaatacaaaaattagctgggcatggtggctcatgcctatagtccctgctacttgggaggctgagacaggagaattgcttgaacccaggaggcagaggttgcagtgagccaagatcacgccactgcacaccagcctgggtgacagagcaagactccatccccctgcaaaaaaaaagaaaaagaaaaagaaaaaagtatgtgattctacattggcaattttttttttttttttttttttgagacagagtctcgctctatcacccaggctggagggcggtggtgccatcttggctcactgcacgctccgcctcccaggttcacaccattctcctgccccagcctcccaagtagctgagattacaggcacccaccaccacacccggctaatttttttgtattttttagtagagatggggtttcaccatgttagccaggatggtctcaatctcctgacctcatgatccgcccacctcggcctcccaaagtgctgggattacaggcatgagccaccgagcctggccactttttttctttaaatgcttttaagatgttcctactatcttcttgtttttaattaattaatttattattattattattattattattattattatttttttttttttttttttttttagagacagggtcttgcgctgatgccgaggctggagtgtgctagtgccatcgtagctcactgcagtctcaaacacctggtctcaagcaatcgtcctgcctcagcctcctgaggaactaggactagaggtatatactaccatgcccagccaattttaaaaattttttgtagaggtggagactcgctatgttgaccaggctcctctcgaactcctggcctcaagcaatcctcctacctctgcctcccgaagtgttgggattacagggattacaagtgtgagccactgtgccagtccccactgtcttctggcttgcatcgtttctaaaagaaacttggtgtcatccttatttttgtttctctacatgttatatgtcctctttatctggttgctttaactttatttattaattttagtttaatttttaattgacaaataataattgtatttttatggggcacaatgtgatgttttggtctatgtttacattgtggaatgtgtaaatcaagctagtgaacatatccaccacctcacacacttaccattttttgtgtgtggtgagaacatgtaaaggctgctccttgaggccaggcccaatcccagcactttgggaggccgaggcgagtggatcacttgaggtcaggagttcaagactagcctggccaacatggtgaaaccccgtccctactaaaaacacaaaaatcagccaggcgcggtggtacacgcctatagtcctagctacttgggaggctgaggcaggagaatcacttgaacccaagaggcagaggctgcagtgagccaagatcatgctactgcactccagcctgggcaacagagcaagactccatctcaaaaaaaaaaaaaaaaagtctattccttgagcaattttgaaatacacaatacatcattgttaattatggtcaccatagtgggtagtagatcactaaatcttattcttcctgtctaactaaaacttttttccttttgaccaacatctccccattccctccctcaacctcagcccctgataaccaccattccactctctactgctatgagtttgacctttttagatttcacatatgagatcacatggtatttgtctttctgtgcctggcttcttttacttagcataataccttccagatttacccatgttgttgcaaatggaatttccttcttttttaaggctgaatagtattcgtgtgtgtgtgtgtgtgcgtgtgtgtgtgtgtgtgtatcacattttctttatctcttcgttcattaatgatcatttaggatgattccacatcaggctactgtgtatagtgctgcagtaaacatggaagtgtagacatctcttcagcatactgcttccaatctctttggatataaacccagaagtgggattgctggatcatatgtagtgctatttttgtttttttgaggaacctccatacttattttgcataatgctattctaattcacaatactaccaacagtggacatgggttcttttttctctacatgcttgccaaccacttgttatcttttatctttttatatatctggctgcttctaaatttttttctttcttaccaattctgaaccatttgatggtttcttcctttatgctccttgtgcttgaggttcattgagcatctgggatcagtgcacttattgttttcatcaaattcagaagattaggccattatttcttcaaacttttttgtcgttctctgtctacctttgagagctccaattatacatacattaggccacttgaagttgtcattacagttcactaatgctaagttctttttttaagtcttgtttctgtgtttcattttggacactttctattgctacatcttcaaatttactaattttttcttctgcaatatctaatctgctcctaatcctatccagtgtattttccatattagatattgtagttttcataactagaagcatgatttggttctgttttcacccatgtatctatataacatgtccagtctttcactcagcttcttaaacatttagaatatggtcagaataactttttttgctgttttgttttagagacagggtctcactttgttactcaggctggagcgcagtggcatgatcacagctcactgcagccccaacctcctcgtctcaaggaatcctcccacctcagcctcctatgtagctgggaccacaggtacacaccaccacacctggctaatttttaaattttttgaagagacgggtctcactttgttgcccagactggtctcaaactcctgggttcaaacaatcctccagccttggcctcccaacgtgttgggattacaggcatgagccactgtacccagcccagaataactttttaaaaatgtcttgaggccgaggttgggaaataatctgaggtcgggagttcgagaccagcctgaccaacatggagaaaccccgtctctacaaaaaatacaaaattagccaggcacagtggcacatgcctgtaatcccagctacttgggaggctgaggcaggagaattgcttgaacccgggaggcagaggttgtggtgagccgagatcacaccattggactccagcctgggcaacaagagcgaaactccatctcaaaaaaaaaaaaaaaaaaaactcttagccacaatttctatcatctgtgtcacttctgagtccctttctattcagttatttttctccttgtcatgggtcatatttttctgattcttcatgtgtcctgtaattttcttttctttttttttttggagatggagtcttactctctcacccaggctgtagtgcgatggcacaatcttggctcactgcaacctccacctcctgggttcaagtgattctcctgcctcagcctcccaggtagctgggattacaggtgctcaccaccatgcccagataattttttgtatttttagcagagacggggtttcaccatgatggccaagctggttttgaactcttgacctcaagtgatccgcccacctcggcctcccaaagtgctaggattacaggcatgagccaccgtgcctggccagttgttctcattggatgtcatatgttgggaactttattgggtgatggatatttttgatttcctataaatattcttgaactttgttctgggatgcaattaagttacttggaaaatctttgatcctttcaggtcctgtttctcagcttcattagatgggactatcacagtgtttgttttagagataactttgccccactgctgaggcaaaaccactttgagcttcacctgatgccccatgacttcagtgatcttccactgtgggaggcgagagcaggactatatccagctccatgtgggccccaggcagcgttcactatcatcatttcaggttgctactgaagtatccctttttcaggctctcagctggcagagcaaatacatatatgtatacatactaacctatgtctatacaggaatctatcggtatttctgtctgtggccatctgtagctgtatgaagccaaacatgagtgtgtgctgatgtctccagccctcatctgttaccagatggatcgttctagcctcctccacttgcctacctgtcaattcaccattccttgagttcatggttcattttcagtatacctgcacagtggtatcagaactgttaacccacaccctgtgggaaaaaaactccatcagctagagcacagtgtttacagccagatccttttgcctttagtcttacagattccaatcattccaaattattcggtgcagcgcctttccgcacctgcacccactttttcccctgagattgtttcctacattcgtagcacagttagattgttttgttacattctgcatttcaccctgggatcctccaacctcctaagttatttttgttttatttgcacacattaggttcaatctgaactataaagttctgtgggttttcacaaatgcgtagtgtcatgtatccaccactacattttccttctctctctttcttgctttctcgccttcttgtcttgctctgtcacccaggctggagtgcagtggcacaatctcggctcactacaacctccgtctcctgggttcaagccattctgctgcctcagcttcccgagtagctgggactacaggcacgcaccaccacccctggctaactttttgtatttttacaaaatacaaaagacgatgtttcactatgtgggccaggctggtctcgaactcctgaccttgtgatccacctacctcggcctcccaaagtgttgggattacaggcgtgagccaccacacccggtctctctccttcctttcctttcctctcctttccttttctttctttctctttccctctcctctcttctcctctcctctcctttgatggaggtctcactgtgacacccaggctggagtacagtggcagcataatctcagctcactgtagcctcagcctcccagggctcaggtgatcctcccacctcagcctcccaagtagctgggattacaggtgcacaccgctgagcccagcaaatttttgtattttttgtaaagatagggtttcaccatgttgcccaggctggtctcaaactcctgagctcaagttatctgccagcctcggcctcccaaagtgctgggatgacaggcatgagctaccgtgcccagaccactgttagattttcatatgaatagtttcaccacatcaaaaaaccccatgcttcacctattcaaccctgcctctcccacccccagccagctcagaaatggttctttttaccattgctataattttgccttttccagaacgccatgaatttgaaatcatatagtatgtagccttttcagactgacttctttcatagcaatatgcatttaagagtcatccatgtctttccatggcttgatatctcatttctttttacactgaatgagttcccactgtctgtttgtaccacagtttgtatatctattcacctatctaagggcatcttggttgcttccaatttttggcaattaataaagctggccatgcacagtggctcacacctgtaatcccagcattttgggaggccaaggcgggcagatcacttgaggtcaggagtttgagaccagcctggccaacatggtgaaacgctgtctctactaaaaatacaaaaattagccgggcgtggtaatgggcacctgtaatcccagctacttggaaggctgaggcaggagaatcacttgaacctggaggcagaggttgcagtgagctgagatcgtgccactccactccagcctgggtgacagagtgagactctgtcccaaaaagaaaaagaataaactgctgtatacatgtgtaggttttgtgtggacagaagttttcaaatcagttggacaaatacctaagagtgtgattccatcatacagtaaaactgctttgctttgtcagaaactgccagaatgtcctccaagggggctgtctcatgttgcattcccaccagcaatgaatgggggttcctgttgctccacatcctcaccagatttgatgatgtcagttttgtggattttagtcatcctagtaggtgtgtggtgacaccacattgttgttctcattctcagtgccccgatgacatatcatgctgagcattgtttcatatgcttacttgccatctgtatatcgtccttgctgaagtgactgttcagatgttcagatcttttgcccattttctttctttttttttttttttttccttttgatacggagtcttgctctgtcgccaggctggagtgcagtggcacaatctcagctcactacaacctttgcctcccgggtccaagcgattcccctgcctcagcctcccaagtagctgggactacaggcacgcaccaccatggcaagctaactttttcttttttttttcttttcttttttttttgagatgaagtctcgctctgtcacccaggctggagtgcattggtgcgatcttggctcactgcaagctccgcctcctgggttcacgccattctcctgcctcagcctcccgagtagctgggactacaggcgcccccaccacgcccggctaatttttttgtgtttttagtagagacggagtttcaccgtgttagccaggatggtcttgatgtcctgacctcgtgatccgcttgctccggcctcccaaagtgctgggattacaggcgtgagccaccacgcctagcccccatttttcaattgagttgtttgttttaagacctctttgtatattaccacatgtgtattgaaaatattttctcccagtctgtggcttgtctttaattttcttagcaatgtcttttgcagagcagaaggtttcattagctttcatagattccaacttatattttctctttcatggattgtgcatttggtgttgcccacacagatttttatactgtattctggtgccatttactgagttaacaattgcggaagaactggaagaaaggaagcaaacaaaacgagttctgcgtggcactgtcagtgcgggggcatggggagtcctgcagggtgaggtatgggcggtatggcaaggcgcgggcccatagatgtgcaggtctggagatgtgtgcagcggagatgtgcgggcccgagatgtgcgggtccgatgtgtgggtccggagatgtgcgcgtacccagaggtgcagatcggaaatgtgggggtccggaggaaatgtgcggatcaggagaagtgccagtcccgagatgtgcggatcggagatgtggagggctaggagatgcgtgggtccggagatgcgcagatcaggagatgggcgaatcggagatgcgcgggtccggaaatgtgcagagcggagatgtgtggatcaggagatgttggggggtcaggagatgcgggggtccagagatgtgggggtccggagatgtgcgggtctggagatgtgcagagcagagcaaagatgagctgatcggagatgcccaggtccggggatccacgggtccggagacgcgcgggtccggagatgcgtgggtccagagatgtgcgggtccaaagatgtgcaaatctgaagatgtgtggatgggagatgtgcaggtccggagatgcgcggggcggagatgtgtggatcggagatgctcagatcgaagatgtgggaatgaggagatgtgcggggcgggatgtgtggatgggagacgcgcgggcccggagatatgcggggcggagatgtgcgggtccagggatgtgtgatctgaggtgtgtgggtccggagctcggggtcagctcagcagcagtgagagcgagcatgctggctttgggagcacagcacaatggcagctgtaggagtgcaagagggtgtgacccagaggcagggcccggccccgcatgggtgttctgaggtttatgcctcagcactagaagcctcgtatgcgaaatcacatcctcatagacccggttcagacacaggatagtgatgcctggactattcatccgtctctcctctttttccccagacacgctttcaccagcttcgagcccctcctcggtgacttatcctgtggtccccggcagcgtggacgagtctcccagtggagcattgaacatcgaatgtagaatctgcggggacaaggcctcaggctatcattacggagtccacgcgtgtgaaggctgcaaggtagaggggagctggaacagggcctggtggccgccaccatcaactacttatggtcacttttatagcaaatggcagtcattactgagagattgcagaaagtcccggataagaaactgacttcaggccaggcgcggtatctcatgcctataattccagcactttgggagaccgagatgggtggatcacctgagatcaggagttcgataccagcctggccaacatgatgaaaccctgtctctactaaaaataccaaaaaaaattagccaggcgtggtggtgggcgcctgtaagcccagctactcgagaggcaaagacaggagaattgcttgaacccaggagccagaggttgcagtgagccaagattgcgccactgcactccagcctgggcaacaagagtgagactccatcttaaaaaaaaagaaagaaaaaaagaaaaagaaaaagaaactgacctcagtgatagattagcctctctttatagcacagaacccctgagagcgtaagccctgttgtgaactgcgtatttgaggaatctagcttgtacgccccttatgagaatctaatacttgatgttccaaggtggaacactttcatcctgaaactatccctccccacccccatctgtggaaaaattgtcttccatgaaaccggtccctggtggcaaaaaggttggggattgctgctttagagagtctaggacaaatggttcctctgtgctttgtaaatacttagagaagtgcattctttaaaagaaaataagtcacattggaccgggtgcagtggctcacgcctataatctcagcactttgggaggccgaggcggctggatcacctgaggtcaggagttcaagaccagcctggccaacatggtgaaaccctgtctctactaaaaatacaaaaattagccaggtgtggtggtgggtgcctgtaatcccagctacttgggaggctgaagcaggagaattgcttgaactcaggaggcggaggttgcagtgagctgagatcgagccatttcactccagcctaggcgacaagagtaaaacttcatctcaaaaaaaaaaaaaagagagaaaagaaaataagccacattaagaacatcacttcattcgaatacaagacagagagctgttaccgttgatctctggagcctccctgaaggccaggtggggcaggtgttctcatgctcctgccagggaaattggccatcagagacacagagtatcttgcttagggtcccacagcccccagcagcagggactggaaccagagactggctgctcctgctccccagcagttccttcctgcacatcaggggcttctccacctgattcaagcgacaggaaccccctgtgcatcttcatcctcctgctggctcagcctgccctaaacagatgtgacctgggccaggagtgcatgaaggcaggccctgttgtcctgcatgctgccagctggactggtggcccttccgtgtttgtcagcgtggtgatgaggagagctcctgtagcagcgtccctttagggttgcacagacgtgctcaagtctggcgccttatgtacgtgatatgtgggagatcatcatctgaatgtttggtttgaatcagaaatcccttctcacggtgcacgctgcaggtgttcactaacttggaaaatgccaccgcctttctggcacaatgtaccatcttggaacaccagcattctgccctgagccaggcctggcctcagaggcctgggccacagggagaacctcacagccaggacactgtggcactctgctgtctagaagcctgtctccccacccttcccattctaaccccatgcgttcctcagcctccccactgtgcaagcctaggtaaggacattatgaagacgtcagcctgcctctcacattcccctgcacactgctgtccctctcccgcgggccaagcagacccactgtggcaaaaatatagaagaatgacttaaaagcaaagagaaaaaagaacccaaagcaaaaatgaactccttcgcatgttttctaaccatatacctttgaaaaagctccttataaagtggccttttccttagggccatgattaattattcatttagttttgttttttatggactatttagtaacattgtttcttgctgggtagagtttaagatgcttttacaaagcaagaaaattgtttacaaacagctggcttccttttattataatttttgtctttgagggagttaatatactcttacaaaaattcttagaaagtctttagtcacaaatatggaaatgtcacaatgctggggatagttacattcatatacattgtaacaaggctgagtaactctttggaaaactataattgtgttttcccaagtcagatgagggcattttgaaatgacttcgaatgctgcctcattttattgtttttcacattaaatgtaacgacatttaaagttctgtatttgtcctaatcattccagacttcttagaagaactatttctttctttttttttttttttttttttttttttttgagatggagtctcactctgtcgcgcaggctggagtgcagtggcacaatctcagctcactgcaacctccgcctcctgggttcaagtgattgtcctacctcagcctcctgagtagctgggactacagacttacatcaccatgcccggctaatttttgtatttttagtagagacagggttgcaccatgttggctaggctggtctcgaactcctgacctcaggtgatccacccgcctcagcctcctaaagtgctgggattacaggcatgatcaccatgcctggcctggaataacttttctctaaattttgttcatttaaaaagaaacaataaatgagcaacaaaaaaggtgagtaaagcaagtgcgctggtttctcagtggcccaggtctttaaatccactgtgtattaccctcacagggcttctttcggcgaacgattcgactcaagctggtgtatgacaagtgcgaccgcagctgcaagatccagaaaaagaacagaaacaaatgccagtattgtcgatttcacaagtgcctttctgtcgggatgtcacacaacggtaggtaaggtggccctgcacattttcccagttcgttcctcagttccccttccttgctccaagggaacagatcaagctatggatgaatgtgcttcaacatttcacacccaagtcattttgtaatcagagtggcctaagaaaataaaagtcgcccaggcgcggtggttcacgcctgtaatcccagcactttgggaggctgaggtgggtggatcacctcaggtcaggagtttgagaccagcctggccaatatggtgaaaccccgtctctactaagaatgcaaaaattagctgggtgtggtggcacatgcctgtagtcccagctactcgggaggctgaggcagaagaatcgcttgaacccgggaggcggaggttgcagtgagctgagattgcgccactgcactccagcctgggcgacagagggagattccgtctcacaaaaaaaaaaaaaagaaaaagaaagaaagaaagaaaataaaagtctcccaggtgcggtggttcacacctgtaatcccagcactttggaggccgaggcgggtggatcacttgaggtcaggagtttgagaccagcctggcgaacatggcaaaaccccgtctctaataaaaatacaaaaattagctgggcatggtagtgcacacctgtaatcccagctacttgggaggatgagacaggagaatagcttgaacccgggaggcggaggttgcagtgagctgagatcgcaccactgcactccagcctgggcgacagagtgcgactccgtctcaaaaaaaaagaaaaaaaaagaaaaagtctcaaatagctgagattcagtggtgcattggactcgctgttagaaacttcagtggtaagactttgatacagaatcgaaaaaccaagtggaaggcaccaaaatgacagaatgttcacctcgtccataggaagggtgtaccacctcaaacatctcaccacgttatgaatttccttctagccaatcatttaatagtttcagaacatgctaattgtgatgtgaatgtaagtcgttcataagagttgcatgtctaccttctggaaaaagaagcagttattatataaactcatcccgaagccccgttcacctccttcactcaaaggttgatgatgcacctgatagtggtgtgcaccctactaatgagacgaacgatggtgtcaccttcagcctgcacctgttaacgatggtgtcaccttcagcctgcacctgtttaaacatctacagtgtatggagtttgagtttttcatctctccatagtggaaagccgaatagtaatgaaggatgggtctgaactgcctgtgaattttcattcctggtttaaagtcctgggggagcccctcgtccagccctgtccgcgcagtcatgacctcactgctcatgcctgtgtttccccctccaaaccctagcgattcgttttggacgaatgccaagatctgagaaagcaaaactgaaagcagaaattcttacctgtgaacatgacatagaagattctgaaactgcagatctcaaatctctggccaagagaatctacgaggcctacttgaagaacttcaacatgaacaaggtcaaagcccgggtcatcctctcaggaaaggccagtaacaatccagtaggtgtttgcggctgttctgggttctcttggcaacatggaaccagtgtcgtagaggacgattaaggacacatgtgttgaatgttgagaaaattatatttatcccacagttaagcaaaggacagcgaagatggaaacagttcattctgagactctgagctgtagcttaacaacaactcctttcttcttgcttggagccacctcaaagctcttagcaactaagttattatactggctatgtaattaatacacttaaaaaaaaccttaatagcttaccaagtactaagatgatttcttaggagcattttttcttaaatagagataggttcttgctctgttgcccaggctggaatgcagtggtgcaatcatagttcactgcagccttgaactcctgggctcaagcaatcctcctgcctcagcctcccaaggagctgggactacaggtgtgcaccaccacacctggctatgtttgatgttgttgttgttttgttttgtttttgttttttggtagagatgagatgtttcccaggctggtctcaaactcctggcctcaagtgatcttcccacctcggcctcccaaagcactggcattacaggtgtgagtcatggcacccagcattaactggatttaaaaaaaaaaaaactgaccaggcaagatgggtcatgcctgtaatcctggcactctggggaggccaaggtgggcagattgcttgagtccaggagtttgataccagcctggccaacatggagaaaccccaactctactaaagatacaaaaattagctgagcagggtggcacacacctgtaattccagctacttgggtggcttaggcatgagaattgcttcaacccgggaggcagaggttacagcaagctgagatcatgccactgcactccagcctgggtgacagatcgagaccctatctcaaaaaaaaaatagaataataaaataaatccctactttgaggtgtattagtctgctataaagaaatccctgagacctggtaatttataaagaaaagaggtttaattggctcgtggcccacaaggctgtacaggaagcttctgcttctggggaggcctcagggaatttgactcatagcagaaggtgaagtgggagtaggcgtcttgcatggcaggagcaaaaacaagagacacacacttttcacccatcagatcttgtgagaacgctatcactagagtagcaccaagaggatggtgctaaaccattcatgaaggatcacccccatgatccagtccctcccgccaggcctcacctccaccactggggattacagttcaccatgagatttgggtggggacacagagccaaaccatatcataaggctagaaaaggaaaccacttacttcccactcaaaatgtgctcttggtcctttctcctaaaactactccctccctctcagacaaacatgcctacattctttttccgccttcagtgaaaagacagtgacatcttggggcttagaaagggccacttgtaagccaggcgtggtggctcacgcctgtcatcccagcactttgggaggccaagacaggcggatcacgaggtcaggagatcaagaccatcctggctaacatggtgaaacaccatctccactaaaaatacaaaaaattagccgggcgtggtggcgggcgcctgtagtctcagctacttgggaagctgaggcaggagaatggcgtgaacccaggaggcagagcttgcagtgagccgagatcgtgccactgcacttccagcctgggcgacaaagccagctgtgtctgggcgcggtggctcatgtctgtaatcccagcactttgggaggctgaggtgggtggatcacttgaggtcaggagtttgagaccaccctggccaacatggtgaaaccccatctctattaaaaatacaaaaaattagctgggcatggtagcggttgcctgtaatcccagctacttgggaggctgaggcaggagaattgcttgaacctgggagctggaggttgcagtgagctgagatcgcaccactgcactccagcttgggcaacagagtgagactctgtctcaaaaaaaaaaagaaaggaaaagaaaggaccacttgttatagaaagcctgtcttttaaggtagctctggaccttttcagaggcagccaaattgcccctcatggttcgtcccccacatccccgcctgcctggcctaagtcctccttccccctccccaacagttaaataagtctttgtctccattacaaaacaaatctcagagctaccttcaaagaagagccagccctcagttggtgaatgaagatactttgacattttcctatgagcatggtgaaacaggtttaatttgtattaaatagcttgaagcaatccttattgggaattacaaggtggaattttagtcacaggaaaataaagcatttcacaagctacttactttcatgaacaaaccaaacctcttctttactgagtcctttaattcttcagtgaattctccaattaaataggccgagacattttagaagtttccagcagacacccacactaggcagctccagaggcttgtcccaattagaactttcctggattacgagagtgaaagaaaaggtaacttttagcttcgagtctctatcctggatatgattagtacagcccaaaattgggatggctaaaacttttgtttgccagcttatatttctcccttggatttcagaattgaaagcaggctgggcacagtggctcacactgtaatcccagcactttgggaggctgaggcgggaggatcacttgaggcaatccaagagtttgagaccaggcaacacaaggagacctcgtctctacaaaaaatgattttttaaaaaactagctgggcatggtggcatgtgcctgtggtcccaggtacttgggaagctgagatgggaggatggcttgagcccaggagttcaaaaccaacctgggcaacatggcaagaccacatctctacaaaaaataaaaacattatccaggcatggtggcacatgcctatagtccccgcgacttgggaggttgaggaggatgccttgaggccaggagttcaaggctgcagcgagccacgatcgcgccactgcactccagcctaggcgacaaagcgagactctctaaaaaaaattcgaagcagagttaagttgtctttcttcctaacaacctgcccccaccatggggtgcgaatgggactcctggagtcctcctgcacctccccttggagaccaccaagctctaggaaccccatcaccctcagctgagggtcacatgcagcaactagcaggcgggaatctgtttgcattttggccttaaagaaataaataataggccaggcgcggtggctcatgcctgtaatcccagcactttgggaggctgaggcaggtggatcacctgaggtcaggagttggagaccagcctgaccaatatggtgaaaccccgtctctactaaaaatacaaaaattagctaggcatggtcgtgggcacctgtaatcccaactacccaggaggctgaggcaggagaattgcttgaacctggaaggcagaggttgcagtgagccgagatcacaccactgcactccagcctgggtgacagagcgagactccatctcaaaaaaaaaaaaaaaagagggccaggcgtggttgctcatgcttatgcctgtaatcccagcactgtgggaggcagaggagggcggattacctgagctcaggagttcgagaccagcctgggcaacatggtaaaaccccatctctactaaaatacaaaaaattagccgggcatggcagtgtgcgcctgtagtcccatctattcgggaggctgaggcaggagaatggcgtgaacctgggaggtggaggttgcagggagccgagatcacaccggtgcactccagcctgggtgacagagtgagactccatctcaaaaaaaaaaaaaaagaaagaaatgatagatgaatagtttaggattggggttcacaatttggttttctgtagaaaaagagaaccgggcactcttccgagagtcagatgccctcttccacccacacccacaaagccagagcaccgcaggtaccagttttcaaggcaacctccaaccatcatgtgactctttgtgtttgatcacactgtttgctccaagccagggttgcgtcccaccccatgtccttgtctgcgcacgggacgctggaggcacggccccctcctccctgcctagcctgctgacgggctttccagagctggctccttcaggtgcaggataccctctctgcttagtctgggaaaaggccccgttggcaggatgcccaccaccaggccacactgcctgaatctattggcagagctctggttttgtggccaaggtgggtagtggaagaccatagcctgtgtcccttacacatctcagaaagcaaccccatctgtgggcaagaaatctgttagggagaccaagcagcggcctggaaacaccttgatctctgcccagtggcccacatgcggtcgccgtttcatcagtttccagcctgggtgacctcacagccccagccacgccccacagagcctcaggaaggcacactgacctcagggccggcggctgacttcatttctgtttggggatgagaggcggcacagtaaactgtccaggccagtaaactaatggattcatacgaaccgtaatgaacgtgggctgtgtgctggggaaggcaggctcgcctcctccctgcaggggctgctggggtgaaagcaaccctgaaatgttcaaagccttgatggggaagcacgggggatggatagattttaatttcaaagcagccctctggtttgctataagcgggggactgaatttctctttgcagtggccaatgcctttcttctgtcaagatcagctcgtggccttcagatcagatgacgcaaagccccatggctgagctggaacaggctagaatgctgggggggggcctgaaaccggtgggggagttgtgggaggcctagaatcagccaggaggcttgggtcggggttggaaccggccagggtgcacggaggaggctgtgggggcagggggaggccgctgcatggagccgcatagatgccattgcttgaggaaaggtgggctttagctgagggaaggagtgaggggtggatggagaatgtctgtgtccatctggacactgggactgtttgagcccctgagatttcagaaccgtgggccagaaaatggtcagggcccttggtgatggggaagggcgcctctggggaactcactgccccttgatttgagggtaacagggatggaagcagagtcagggggctgagggaggcaataaaaatgggtgcttttcaacagtgtctaaaaacataagatgttgacctgtcaggggttgagaatgtcgtcagaagactttggaggaagcaacagaaaatgagactgaggggcttgggcagagtcagtgccttctgtgtgatgcacgctcatgcacaaatgcacgcacatacccacactcacacatccgtgcacacacgggtacacacacatacacgtgcacccacatgcatgctcacacacatgcacccacagtcacacatccatgcatgcatgtgtacacaaacacacccacacatacacatgcacccacacgtgtacacagatgcacctccacccccatacatgcacatggacacacacatgcacccacacgcacacaagcatccatgctcacatgggtacacactcacacatccatgcatgcacgtgtaaacacacacacccccacacatacacgtgcacccacacatgcacacagacgcacctccacccccacacacgcacacacacacatgcacccacacatggatacacgcacactcacacatgtacccacacctgtgtgtacacacacacatgcatgctcacacacatgcacccaggcacacacaaatccacattcacccatacagtcacacacatgcatacacacacatacaaacacatgcattcacacagatgcatacacacacacacttacaaactacacatgtgcttatacatgctcacatgcatgtatatgcacacacataccctcaccttatgcacacatgtacccacacacgtacccacacatatacaagcatgcacacatatatatatatacacatgctcacacgcatacccacactcacatgtgtgcacatatgctcacacacacgtgcacacacatgctcacacacacacttactgttgctcaggcttagctgctttgggcttaagaagcaaactgcaccttccaaaaaatgagtgtggtgttcagttaaacaaccaaataattctttagcactgaatatgtggactttagaaattcaaactataaggtgataataacgttgtcctgctactttttaatctaacaaacatatcagaactgacactcagttcaaatgaagaaagtaggaattgggcgtgccgtgttattttttcaaagattctcctattgctccaaattgttggggattatcttaaagtctttgaatagcttcagttatggaagattttaccctctgagaatagaactgaattttagacaaaccatgagtccattgtagctagactggcatgcaagttgggattaaacagagtaaaacgtcttgtttaaaaaaataagaaaggccggcttgggcaacatagtgagacctcctctatgaaaagttagctgggcatggtggtgtgcgcctgtggttccagccgctcaggaggccgaggcaggaggatggaggtcaagactgcagtggactgtggttgcgccactgtactccagcctgggtgacacagcaagaccccgtctcaaaaaaagaaaacagaaaaaagaaaaaaaaagttgagcaaggagactaatttgtgacatgcagctgaacatggtttttaagaccagttttgaaagaggaattccaacattattcttaacatttcagaagcctgggcataagggtgacctccagggtgccgtgttataacaggactgctcctttcaacagctatgaccttataccatgtcttggggtgttgcctgccgtgtgacagtccaatattatacctactacttaagttttctttagattaaaaaatgtgcttcatattttatgccatttctacaaatgtatagtaaaacataaccaagagagcttattaaataatttcatccaaagcagttctaccagtgcttcacatttattttttatttatttatttatttttgagactgagtctcactctcttgcccaggctggagtgcagtggcgcaatctcagctcactgcaacctccccctcctgggttcaagcgattctcctgcctcagcctcctaagtagctgggattacaggtgccagccaccacacccgactaatttttgtatttttagtagacacgggcttttgccatgttggccgggctggtctcgaaatcctgacctcaggtcatccacctaccttggcctcccaaagtgctggcattgcgggcatgagctactgcgcctggtccacatttaattttttgcaaaaagatgacagctgctaacagagatgaattctcatgagtgatatcattgagcttcgtaggccacatgagtgtgtgccgggaccagtgtggcagcaagcggggcgttctgctctcggcatggagtgattggggaaaatctaggcagcttcctgcctcacgctgtttaaaacctttataatgtgctttatttcatttatttgaaatgactgcctgtcgtgtcagatatattcatagtcaagcttgagtataaaaggcatattccaaagttaaatataagctgctgcatagatttttttgtaaaatgatctcaccaagaatgtttatccataaagtttagcgaatttgcaagtgtgtttttcaacagcatttctctttagctttaataaacattggtttcttcatggtaccactcattttgaattcagtggtctccagttctccctgctaaatgaggcccactttctaaaaccaaagtgataattttataaaaatgaaatgagatatttgttaccacagaagtcctcatttacgagagtacatccccatagaactagtccacggtgagcctcaggggcatgcaagctgtttaacgatgcccccagcctagaaaggcccaggcttgggtgttcatgctccgctgttgccttcttgaaattcataatcatctttgaacaaggggtcccgcagtgtgtggtggctcacgcctgtaatcccaacactctgggaggctgaagcgggtggatcacctgaggtcgggagtttgagaccagcctgaccaacatggtgaaaccccatctctactaaaaatacagaaattaaccaggcgtggttggtgggtgcctgtaatcccagctactcaggaggctgaggcaggagaatcactcaaacctgggaggtggaggttgcagtgagtcgagatcacgccactgcactccagcctgggcaacagagcgagactccgtctcaaaaaagaaaaaccaaggggtcccacatttgcatttttgctctgggtcctgtaaattacgtagccaggcctgcatttgtcctgggagatgctctaccaaaaaacaataaataacaccaagcattctgtaatcaaacactgtaggaacccctgcttatcctagcctcattctcattctggaagactgcacatttatcatgttaaagactcagctagggaggcccaacttcattcaactcagtgtttcttatttttttaaaacagaactcattttttaaaaaaattattggctgggcgtggtggctcacgcctgtaatcccagcactttgggaggctgaggtgggcggatcacgaggtcaggagatcgagaccatcctggctaacacggtgaaaccccgtctctactaaaaatacaaaaaaaaatgagctgggcatggtggcgggcgcctgtagtcccagctactggggaggctgaggcaggagaatggcatgaacccgggaggcggagcttgctgtgagccaagatcacgccactgcactccagcctgggcaacagagcgagactccatctcaaaaaaaaaaaaaaattatttaacacctttatttctgctgaatgtactttagaaagattgagtgatttgaataaagtgacggtggcctaagagtctattttctggaattgagggaatactgccatcgatccttgaaaaatatttatttagttcctcctagaggccgggcacagtggctcacgcatgtaatcctggcctgcactttggaaggctgaggtggacagattgcctgagctcaggagttcaagaccagcctgggtaacaaggtgaaacccgtctctactaaaatacaaaaaattagctgggcgtggtgatgtgtgcttgtaatcccagctactcgggaggctgaggcaggagaattgcttgaactcaggaggcggaggcagaggttgcaatgagctgggattgcaccactgcactccagcctgggcaacagagcaagactctgtctcaaaaaaaaaaaaaaattatctagcccctcctagaaatgttaattccttaaatctgagcttcagctttctgtgaagcagaattatctccaaactttaacaaacaatggtcagaactgtttttaaggtcttggagagagatcattttcagtctttattaatcggacttgagattatttagaaacttggctctgaatattgtattcagaatgttttcactcatttgtgagtaattttttaaatatcccctttcctcagatgcagaatcagggctttttgtccagcattatgttgcaagtcctggttctgttgaaacattccataccatctgtgtgatggttatcggcacctccaccggtgccctgaagacagttttgtgctgtgagtccagaaacaggaaacacttcaggctgtgtgtcagaagcattgtcagtggttgtgttttgcccactggcagggggcattctttaaatcctgggatgcttctgcgctttgggctccactgttccagcagtgattagaaataacgctgtaggccgggcgcggtggctcacccctgtaatcccagcactttgggaggctgaggtgggcagattacctgaggtcaggagtgcgacaccagcctgaccaacatggtgtaaccccgtctctactaaaaatacaaaattagctgggcgtggtggcgcatgcctgtaatcccagctactcagaaggctgaggcgggagaatcgcttgaacctgggaggccgaggttgcagtgagccgagattgtgccattgcactccagcctgggcaacaagagcaaaactctgtctcaaaaaaaaaagaaataacaccttagcccactgcattattgacctgtgtctgcatgagctgtggaccacattataatcagagagatctctcagatgttgtcactttcctgctctacccgcagatgtaaatttcagccaacagcagtgtttgtgctcattttccccggctctcccacacatgtaatcccttctgagcatgttggcttcaaataatatggccagccacctcttccaccacgagatcttcaggaaatggcaggccactgggtttacatgcagatggcatgggagcacacaaggcacggctgtggggagttggcacttgctccagaatatggagcaccgagtgaaggtttcagtttcctgcactgagagaaacaagggcattccgaggcttttccactttatccctaaagagtttcacaacgcttgtttgccgatttctacatagatgccacctttctgagttgtatgtatttacatgccaaatgtattcattgagcagcgttaaataatggtgttcacccctaaagtgcatatactggtaaaattaagaatgatcgtaattaagcctcttgcaatagtcattagttcagagaatatttaagaatattaaaggtgctttgctaatgtcctcgttagttttgttttgacaaaatcagtacttcagtttcttgtttcttttttttttgagacggagtcttactctcgctctgtcgcccagactggagactggagtgcagtggcacgatcttggctcactgcaacgtccacctcccaggttcaagcgattctcctgcctcagcctcccgagtagctggggttacaggcacacactatgcctggctaattttttttttttttttgagacggagtctcgctctgtcacccaggctggagtgcagtggcgcaatgtcggctcactgcaagctctgcctcctgggttcacgccattctcctgcctcagcctcccgagtagctgggactacaggcgcccgccaccacacccagctaatttttttgtatttttagtagagacggggtttcaccatgctggccaggctggtctcgaactcttgacctcaggtaaaccacccacctcagcctcccaaagttctgggattacaggcgtgagccaccatgcccagcccagtacttcagtttcttagcgatgaaatccacccaatgtcaggcgatgactattattattttactgatttatactgtttgttctctattaatgtcttattttccccaaccgattttgaagttgagtaaggactatgttccgcgggtatcttgagtcctctgaggcactgagcttggtgatttggacgcaggagctgctcattagtgagctgatagctgggagcatagcgcatcccacatcacctgacttaccttggtgtcctcctttgtagccttttgtcatacatgatatggagacactgtgtatggctgagaagacgctggtggccaagctggtggccaatggcatccagaacaaggaggcggaggtccgcatctttcactgctgccagtgcacgtcagtggagaccgtcacggagctcacggaattcgccaaggccatcccaggcttcgcaaacttggacctgaacgatcaagtgacattgctaaaatacggagtttatgaggccatattcgccatgctgtcttctgtgatgaacaaagacgggatgctggtagcgtatggaaatgggtttataactcgtgaattcctaaaaagcctaaggaaaccgttctgtgatatcatggaacccaagtttgattttgccatgaagttcaatgcactggaactggatgacagtgatatctccctttttgtggctgctatcatttgctgtggaggtgagtggttgatttaatctgctggtatcatgtcactgacaggctcctgtcttgaaaaatttgacaatgggaaatccagtaccagcctgagctgttccagtggaggggacactcacatggtgggaagacgtctgacccccagtcactgctgagaattcagtgggaattataacaatattgtataatattatagtatatattgttattatctataaatacatatttaatattatgtaaatgtatgacattttaatcataatattagccaggtgtgggggtgcacacctttagtcccagctacttactcagtagactgaggcaaaaggatctcttgagcccaggagttcaggttgcaatgagttatgaatgcaccactgcactctagcctgggcaacagaacaagacctatttctttaaaaaaaaattatatattttgcacaaatatatatatagagaaaaagaggtcggacatgggcctgtaatcccagccctttgggaggctgaggtgggtggatcacttgagcccaggaggttgagaccagcctgggcaacatggcaagaccccgtctctacaaaaaaaaaaatagaaaaaattagtcaagtatggtggcatgtacctgtagtcccagctacttgagaggctgaggtgggaggatcacttaagcccaggagacaaaggttgcagtgagccaaggtcacgccaccacactccagcctgggcgacgaagaatgaccctgtctcaaaaaaaaaaaaaaaaaaaattatacacacacacacacacacacatttcgtttatattatatctaatattataaacagatataatttatatattatgatattcctgtatatattatataatgatgttgtattcatattatagacaatattgtatgaagtgctatacagatgtcagtatagttgctgtcacagttggttatgttgatgaaaagtatatttcctaatgcaaaatataatatcagtcagcagccaagtggcagtgactgcaaggtttgctttgcccgaggaagcagatcccagggaaggccgatctggtcctctctgtggaagctggctctgcagcctccacatttttggctcggtgtcacgttcctttaaatagccccatctcaggtctaggaaggtcatccacctactgcaaactcggctgaccttacccagggttggtggagacagatggggtctcccacactgcctgcagccatactgcgcctgggggattgactcactgtcagcatggagctgactcagccctaccagccgtgcccgttactgtgtggctgggcacaagtcagatgaaggaagtccttgcgctctggcataaagtgtacaaagacaaagcagttatgcataatttgtcctttagtatggtcaggatgtagcattgtgggtaaaatgcagttgcagaactatttatatgtagcatgatcacagttttataaaggaaattataatcctatatcaatcctatgtatatagaaaaatgtccagtgagatatatgttaaacctattatggtgggattaaaattatgaggggggatttctatttttcaaaagattcctccttttttttttttttgagacagagtctccgtctgtcaccctggctggagtgcagtggcacgatctcaggtcactgcaacttccgcctcctgggttcaagtgattcgcctgcctcagcctcctgagtagctgagattacaggaacatgccagcacacctggctaatttttgtatttttagtaaagatggggtttcaccatattggccaggctggtctcaaactcctgaccccgggtgacccacccacctcggcctcccaaagtgctgggattacaggcatgagccactgcacccggcaataattcctctctttagagacttaatagttatagccccagccactctggaggccgaggcaggaggattgcttgagcctaggagttccagtccagcctaagcaacagagcaagaccccatcactaaaacaatacaaaaacaagaattttagaaataaaaacttaataattacatttacaaccaaaaacaatgaagatgtttaaatcctcatcactagcaaccctgttaagaatcatagtaatgactgggtctgtaagggagcaccgcctgctgaacatggctcagggcagtattttctggaccaagaatcaggtctcatgctttgagactgtcccaggatgtctagtgccagctaccccaggcaggtcatctggtgtgaatgttgactcttcctgcaccaagtctcagacctgccccaccctcctccccactctgggtctcctgatcttggctcactgcaatctccgtctcccaggttcaagcgattctcccacctcagcctcccgagtatctgggattacaggcgtgagccaccgtgcctggcctacaaaacctagttctaacacaatcactccttaaatatggtggaacacttgaagcttgatatctagtttggattcaaaagcttcatttcccatattatgcaaaactggtggttgtgatctccagaatgtactgttcctcctactagctctaatttttctccctgacaggtggtcatcaggtaaatcacaagtgaaaaggccgcaccataaggtgtacttagggcactattgccgcctagtagtatgaatatttaggaaagagtactggtcctgtctgtccctacttcacctattgactttggaaaaacctatgtctatcttccagtcaagttgacaatatctaaaggcagctcagtttttttctaagaaaggccacataaaataggcatgtttggttcctgaaactgataagcagttcttgggtgattatcacactcaaacctctctctcttctttcgagactagatcgtcctggccttctaaacgtaggacacattgaaaaaatgcaggagggtattgtacatgtgctcagactccacctgcagagcaaccacccggacgatatctttctcttcccaaaacttcttcaaaaaatggcagacctccggcagctggtgacggagcatgcgcagctggtgcagatcatcaagaagacggagtcggatgctgcgctgcacccgctactgcaggagatctacagggacatgtactgagttccttcagatcagccacaccttttccaggagttctgaagctgacagcactacaaaggagacgggggagcagcacgattttgcacaaatatccaccactttaaccttagagcttggacagtctgagctgtaggtaaccggcatattattccatatctttgttttaaccagtacttctaagagcatagaactcaaatgctgggggtaggtggctaatctcaggactgggaagattacggcgaattatgctcaatggtctgattttaactcacccgatgttaatcaatgcacattgctttagatcacattcgtgatttaccatttaattaactggtaacctcaaaattcgtggcctgtcttcccattcaccccgcttttgactattgtgctcctttataattctgaaaactaatcagcactttttaacaatgtttataatcctataagtctagatgtatccaaaggtgaagtatgtaaaaagcagcaaaatatttatttcaaagacttcacttctgtttcctgaatctaaagaaagacaacatgctgctttttaatcataggatggagaattttaaagaactgtttgggccaggcacagtcgctcatacttgtaatcccagcactttgggaggccgaggcgggtggatcacaaggtcagcagatcgagaccatcctggccaacatggtgaaaccctgtctctactaaaaatacaaaaattagccgggtgtggtggcacatgcctgtaatcccagctactcgggaagctgaggcaggagaattgcttgaaccagggagttggaggttgcagtgagctaagactgcaccactgcactccagcctggtgacagaacgagactctgtcttaaaaacaaacaaacaaaaaaaaaatctgttagataagctatcaaaatgcagctgttgttttgtttttggctcactgttttcgtggttgtaactaatatgtggaaaggcccatttccaggtttgcgtagaagagcccagaaaacagagtctcaagacccccgctctggactgtcataagctagcacccgtggtaagcgggacgagacaagctcccgaagcccgccagcttcctgctccactcagctccgtccagtcaacctgaacccacccagtccagctgtctgtgggaatggtggtgttcttagggacagactgacaccttacttgtcagtgttcctccgggccccatttggcagctcccgtatcttttgttatgttgcttttaaagatatgatgttttattgttttaactcttggtgacagtagatgctctctggagcgcagacgaggcacatgtgtcttcatagcctgggctgggtgggagccagtcaccctgcggatcgagagagggggtagagtcttcttcaaatggcagttttacttcaaatggcagatttcacaagagttggttattttttacaatggtttaggttgttaagtctcctttgtatgtaaggtagttttttcaacatctaaaatttttgttttagccttcaaaaccaacttaccaacctcagtccagctgggaaggcagcgttgattatggtagtttgtcaagaatatatggacctggaaacactttctctctctgtccacctggtagataaattgtcctgttgagaatttttagatctggactggaactgccaggaccaccgcctccagggagtcgctgggcacctggaggtatcgtcgatgcctctcccccatctttagaaaatttggctcttctgaggtcattattattttaagaatgattaggattgataagggtcccatgaccagcattatgaaaatgcgagagtgggaaggacacagtgtgagacttccactagaaaaaagtgaaagttagggttaggacatccttttttaaaaattacaaatttagtccgttttggtttttgtaatcaggctaggcacagtggctcacacatggaatcccagcactttgggaggccgaggtgggaggatcacttgagcccaggagttcgagaccagcctaggcaacatagcaagaccctgtctgtacacaaaatttaaaaattagttcatcggggtggcacacatcagtagtcccagctactctgcaggctgaggtgggaggattgcttgaacccaggaggtcgaggctgcagtgagctgtgatctcaccactgcattccagcctgggtgacagagttagattccaccctctcccaccccggcaaaaaaaaaaaaaaaagatgcaatcaaaggggctgttggccagcaatggcagcagcagcggcgggcagtctgcccaagtgtcttaggaaccaaaagcaaataaaagtgtttccatatatgccaccagccaagtggccatcctaattcagaaagaagctagcctttgagtgtctgtcatggtgcatccgtttcagtattatttcctaaaatgagaagcccctgtgtcaacaagatccaggggctggagcccaatgccaagcctgtgttgtccccagcgaccctgcagctgctcgctctgatgtaccctgtgccattcaaggagatgtggtccaggaaagtgagcctcatggttttcagagaagtcattgttctgtttacattttcataaaacctgtttaaaatagctccccgtctcaggctttcagcagtaacagtgagctgactggcaagttcgatgttagctcccgggacactcagcagcgatggtgagcattttggtttccttaaggcccagcaagacttccagggacatctctggtgaagccagaatggagacacccgtgacctcaggctgaaagtcactcgacattggtctcttgtgttgatagggaaggaaatcaggcattcctatttctttaaataacaaaaccactaattgccactcaatgctggaatattttgggtcacctaatcatagatttctcagggcatcaatactcaaatataggctgattatgccccagttcaaatgggaactattaacagagtgcatttcttgcttgctgggtttcaacagacatcagccaaaagaacaaaagagatgtcaggacagattccaggagtgtcggagcacatgtgtggcacccgctccctctggcagcgaatgtaggaagtcgccaaatttacccactcttcaacaagtcattgtttaaacacggtttttcattttctcaacttttaatagcaaaaagtgccaaagtcctcagagacctaacagccttggtctaccgtgctgaccagggtgaaggcacggcgagggactcctcccagacgtgcctcttgtgtgccagctggctgtggctcgggagcagacgcaggcctctccattgtccaggggagcctggcggcgcatccctcctctcccacctcctggcacttccagctgggtgtcccacatgttggattccgtccccaccacacttccagagaccggagaactgtgcagggcctaaggccgtttggatgaattgtcaaaacaagatgcttccagttacagcggcaggagcgggactgggagcacgggctgacggctgctggtgcctttcttcccacctcgcttgcctgtttccgcttgacccttcctccagctccgatgagaagagtataaagcatcttcctaacgggtgtgtttgctatacgaacataatggacgtgaagtggggcagaaacccagaactcagcattcaaggatgcccaggagagctgtccctgttttaaagagctgtgttttgttttgtttcgcatttagagagcagacaaggcacccttctgctgcgctgatacgtttcttacactgggccattttagacccccagggaaacagccttcctggagcgttgtctggaggttccagggacagggcagcctcccagagccgagcaagagctcaaggtacaaatgagagatttgctataccgtgagaagtcaacaacttagccaccacttccccgcaatggaccatgtaacaaatacctcagcaggccctgcaaaaggccatgctagagctgaggcgcacagcctgtggcctctgtagttagggcaggtgggatggagactccttgagtgcacacacctgagcctgcccacacacaggggagcagcatctcgtatgacgtctggaaggaacttcggttgtgtaaagggagccttgaagatacgtgcaaaaggtgctaccccaatttggtgaaactgacattgggcacgtcttgggcttaggagaagcggccgatggtcccggcctgcagtgacaaacccccctccccgcaccgcccccagcaccccctctcctcttcacctcttcctgctggccacgaggaagccacttcctcagagagaccctaccagatgcggatggaaacagatgcaccaaagcaagccctgatgaaaccgcgacttcctaaggtctgtctcctctgaacttgcacctgggcctctctgtgtttggttccaagcacttcccacctcaaactcccattttcaaaccactgtatctctgcgcacatctgctacttaccagccgcatacatgatggagggttttttggtcctgatccagtggccacacctgtctttgaaatgtctcactgaactccagttttaaaatagattcattgcttcaacacagcaagcccaatgcacccagctaagactggcttgaccgacagcctggcctttggtggggggcttcctggggcctggggaaagctggccaccttcaacagctggtacctcttcaacagtgtggcctttcaaaatgcagatgccaccaggagaacatgcccacagctcaccacctatggatgccatggctctgggcagctttcaaagcaggttcctgtggtctcctcagctgtttgagggggtaacagcaaatcagcctccattttaaaatgaaaacaccagcctccagatgtagggcctgctgggtgttgctagccgctggtccccaggcacggtgcactttctccacctcctgcagcctccctgttgtttctagactcttgcacctggtgagtgcaaggataggtgacccaggggcctgcagccttgtcctcagctcccatctcctggactgccagcctcaccctctgcagttagcatggttggcctgatgcagggatcccgagggattactttttagaccttctttcacattcagaaaagtagtatagattcaggagaggcaagaaaattatgctgtccatagaagtcacccatgaagactgatgccaccacctgaaggctcatgattgttaaaaatgtccacgggaacctctcgtccacaggaggtttgtctcaacacttcccatttttacggcattggcattgccaagcatggggaagtatctgctcttctcatgttaaaagtggcccagcttttcttaactcagtccaagctgacttgtttagctgcactggaatttcttaccaaccaaatatttgcatcgagcaaagggggctgtgtgcacctccctaatggcagcgatgatggctgctgtcattcaagcccatcttcagacgtcacagtctggaagtgaaatgtccacaaacatctgtggcagaaaaggctatacggaccacccagttgtgctgcagctttacagagcaaggaagggttgtggcaaataaatgattaacctgcctcgactgtgctgagggcaacaaaggccatctcaccaaaggattattcgatgccattaaatcatcccgtgaccttcctgcttccgagtccatggcctttgcccagggcatgtactcccctgagaggccttctgcctagaaagatctatgactgggttccaaagttgaggcctaggtttttgctgggatttagatattttcaggcaccattttgacagcattcaggaaaacggttattgaccccatagactagggtaagaataaaggcaataaatttggtctgactcagaatataggagatccatatatttctctggaaaccacagtgtacactaaaatgtgaaattgaaggttttgttaaaaagaaaaagataatgagcttcatgctttgtttaattacataatgatttccattacgctatttctgtgaaatgcagcaggttcttaaacgttatttcagtggcatgggctggaagcttatcacaaaaagccatgtgtgtggccttatcagaacagaaagagacaggctggtgcccaaggctgctgcctgctccaccttttgccagctctggacatctgaggacgtcccggcagatctggaatggggccctcaactgaccatttgcttctcagaatttcagtttgagacatgagaggtataatcagttacttttctccccccagagaaacccttttgtgaggggagaggagctatggtatgtggttcagctgaaacacatacaactgcatccttttggagtcctttgccaacaaaaacagaccaacagaccagatggtgtccatgttcaatatcatgtcttgatggacgcagctgatgacctcaaatacttgagtggtctcatggctgttagatggattatttgaaaaaaaaaaaaaaaaaagagagaaaaaataattgatttttacatcagagatagcaaactaagacctggggaggggggtcagcttttattttattttattttttttaagtttgctagttgggtcaaatgtgaggaggagggagtctacctgccacctcttctcttgcccctcttctgcccacacatccagcatccaaaatccattcatttaatgaattgataaagtgccgtgcaaactggtgcacaaacaggcccccagtccacgcagcctggctcctaggaaaagtggtgaccgggcgtgggggggcatgccgcagccctgggacacagtcgggcaccttccccggacccccaggccttggctgtgcctcaagtcagagagggtcagccttcaggccccggagacgagtgactggccgatcatttcacaataaaatcactcacttttggcaacttcactttttttaaggcacagtcagttccttttctcatgtacctcacaaaagatgaagaccatgtagtactctttttggtaaagttacagtgttcatgttaaatatcacttttttctacattgtgtggtaaaaagaactacgttaatagctatatcttaaatactgtgatttgactttttgaaaaatatcctaatacaaatattttactaacttacaatcactcatttaataagaaacatttggattcttttgaaatcagtgttaattgactcatattcttaaaagcctggctcttgaccctattggaaacacaaaggaagctgaaatcaaacatctaaaatacactgcgtacacgtgtgcgtgcacacacacacacacacacacacacacacagctcttcatttctcctgagccatgcagaatttactttcaatgtggaaatctgttccctttaccacactgtatatgcacagagcacaagagaggctatctctagtcacttccaccagcgaggccttagactccgtattagaggccaccgatttcatacaacagtgtttcgctaaagacccttcactattcttgtttagtaaatagctgtctgctcttcagggaactgttacctatgggttattaccaaagaacgctggcaattggaaatgtcctgatggaaattctttgcacgtgccggttctctggcatcctccaggtggcccaacccaaagcagaaagcagaaaccacagaccccgtgagtctccccataccttgtttccaataacttggcaaaacttcttggtgcatattggttacaccctctgggattcataatgccattaggctaaaaccctaagagagagggttgacagaaacacacgcgagaatgaggcagatcccagagcaaggactgggcccagactctccacatgtgctctactagtgagtgccttatactctcagtattttggggcttacagcttcttatttgtgctaaaaaggtgcagttccaaagtaggaactgccacacaggccccagcatcctctctccaacttcatacctctctcctggtggggggagcgggcatccaggacctccggaatcaaggatgtgcagagaagagcgaaagtaatttttctagtcacatgaactgattggttccaggcaattagaaaatggctataaaataaccttaattttaaaaaaaaatcttgggtcttcgttttcctattaggagactgaactgaccacatgtattgatttatatcctgaatatatgggaacttctgtgtttgggatgtcctactgtaagactgatgaatgtacagagttaatttcagggtacagttttgccttaatggttttaaaaaataaactattttttaaaatttt

SEQ ID NO: 3 - DNA, 15496 bp, Homo sapiens
ggctccacccccaagccaggcgaggcaggttccgaggttggaacacctggcgagtcctcggtgtcggtggccggcagtcatctcgcggccgttcaggtgagggggttggaggagtggctcatgagcgaggaagggggagcaggcgggctcccacccggtgctccgtgagatcgaggggagcgggttctgggtgcggatgcacgcgctgggcgggacgctggcagtggtacccgagacggggcggaaggagactggagtgaaggtgggcctaggctaaggtacgtgctagaaaggatgaaaacggagtgaaattcttaagtgatggaactaggctagggcatgtttcttgccctttaaaatgtgttgtcttcgggagacaggacgtagaagatagttgcagcacagggtgataggctggcgaaagttatacaaaagcaggaaccactagaaggaggtaagatgtagtgtgctttgggagtagtggggttgggaagggcgtccgagaggaggttactgaaggatgactaggagttgaatgggaggacatcacctgtaagggaacgatatttccgtgggcagagaggaatgaagcagtagcaaccatgagtgatcagatactgcaaaaatgtgaagtgtaggatggcgagaatgtaagaaatgaagagtgaagaagtctggaagggcctcgtgtgcatcaatcacagcggggcttgatctttatgcttagggcaagcactcccttgaactttgagtgttttaaggaggttatctctgatgtttaaatttatatagatcgtggcattgcatcttagaaataaggtttaggaagggcaagcttggaggcagggcaagtccagaaaatgaaggagctggtgaaatccgtgttaaagtgccaaaggacagagactggctgacagctaaacttcaaggtttctgagaatccacaaataactaaatttatctagtcaacctgttccagaacaggcttccagtcatttaggttgcccaagaatgagtaaaggaaaaggaaattcaattttccaagaccttgtttcccctctcctctttaattccttgttcggttagcaacagtatatccattccctcgctcctttgtgaaaagtaaattcctgaatgttaactaaaccaagtgtttctaaattgggtaagagtttgaagacttaaggcagcagaatgggagagacttaaaacgttatgtctgagaattaggcattaaaggaggcctagtatttgggcgggggttgtgaggagcacatactgaacctttggacctgttgagtgagttcatgtgcctctgaactctctgactggatatgaccagtaaacttggataattagatcctggagtttaggggagagggctagagatagagatgatggatgtcagcatatttttaaaacagaaaatagttaagatcacccaagacaatctggaatcgttagaagggagtaaggaaggcattattgggaaactttccagcttcaattctcatattttttctaatctcctggttgagtctttggagttgctgttctctctatgcaaaacccctcccttgaccctctctccctcactctattttttaatttgtcacctccttctcctgttctaggtctcagtttagatagcacctttctctagaagttcatagcactgtgtattcccccctttattgttcttatcacataatttttgatggtttggacactagttgttattcctcactaaattttatgttttatgaactcaggggtaagggcaccagctagcacaatgaatgcacaatacttgtcagagtgaatgcatttaagttccaagaaccaaggaaaggcggtatttcaagaagagaagtatcaaatcttccagattagtcaaataaactccaaaaaaaaaaaaaaaggtttattggatttggcagctggagatccatagcgatttttttttttttttttttttttttttgagacggagtctcactctgtcgcccaggctggaatgcagtgtcgtgatctctgctcgctgcaacctcagcctcccgggttcaagcaattctcctgcctcagcctccccagtaggtggaattacaggcatacgccaccacacccggctaatttttttgtatttttttggtggagatgtttcaccatattggccagactggtctggaactcctgaccttgtgatccgcccacctcagcctcccaaagtgctgggattaccagcgtaagccaccacacccagcctccttagtgattttagtaagagtaagttcagtgcagtgatgacaatagaatgcagattgcagttgctagaatataaacaggaaataagaagataaagacaactcgtggaataccttttcatagagcttaggtaaactgtaggaattattctccttgtactctaatacttattatgggttttatttataattatagtgtaatataatggatgagtgcatgggcttccccacttagcatttgttaagcattaacttaacattaagcattagactttgggcaagttgcttaatctttctaaacctcagttattttatctataaaatggtgataaaataatacctacctcacgaaggtgtggtaaggattaaagtgaaaatgtagagagcaggtagcatgctttgaacacagttcttggcacagaaagtgcccaataattgttagtttcttgtagctattacatgccaggtcctgtgctaactaagcgctttatatgcattgtctcttggactcattggaagacctactgttttaatttttgctgctgataaaactgcatcacagagaggttacctaatttgcccaaggtcacaggacaggactagtaagtggtcttggttcattattgtcaaatttactaatcaccttgagaaaaattaagattggatggttgccttattttacaacttagaagatgattgaagacattttggtgcaggtggggagccagattgcaagtagctcagtgagttgtgtgggtgagttaagcaaccttttttattctttttttttgagacggagttttgctgttggtgcccaggctagagtgcagtcacagcttactgaaacctccacctcctcatttcaagcgattcacctgaactcctgaccttaggtgatctgcccgcatcagcctccccaaggtgctgggattacaggcgtgagccaccatgcccagctgagttaagcaatctttatgtagagctctcctttgagaaagaagttggttggttcaaagaaagataaatgggacagtggcttggaagaggtaatggaggctaggaaggtgtttatcaacaaaggaagatgtaggctgggcgcagtggctcacacctataatccccacactttgggaggctgagatgggaggattacttgagcctaggagtttaagaccagtctgggcaacatagggtgacccctgtctccacaaaaaattaaaaaaattagccaggcgtggtggcatgtgcctgtggtcccagctacgaggggctgaggtgggaggattgcttgagcctgggaggtcgaggctgcaatgagccataattgtgccactgcactccagcttgggtgacagagtgagaccctgtctcaaaaaaaaagaaaaaaaaaaagaaaagacgtgaatgtgtttttagacctgaaggaatggattccatgaagggagaaggatgaaagatgggaaaggataagtgatggacaagttcttgaggtaagataagaacacaggaagactagtcagtcttagaggaaagaatgaatgagcaaagaaattttaaggcctgtaatgacacaggatggaacactatagtcactgtggtgtaagtcatttgagatgagtaggacagaaggaggacggcctgaagtgaattcagatgcctggaggagttggctaggttctcaatattccttctgtagaatgggataaaaggtcagtttgagaagtgttggggaaggggacttttaaagcactatttagaatgcttctgaggctttaaaatactcatttttaaaatggtccaaaaaattcataaattagaagcagcagtggtgaacatttttaggaaagtgacccttgagaagtttattttttggttagtgacctattgagcttatttattaggtaagtagaacatgctcatttaaaaagtttaaattgtgcaaaagacatatgtcagatttttttttctgtcttccataacactatttcctaccccgccgcgctctgtcttccgtaacactctcccctaccccgtcgccactctgtcttccataacactgtcccctactccaccacactgtctcctaccccgccgagctgtcttccataacactctcccctaccccgccacgctgtcttcattaacactatctcctgccctgccacacaactctgttttcctagaagtcaccagtgtgaatttttccctttatccatatgtacattttttgtttctgtgtgtctgtgtatatacatatgcataaaagtgcatagataaaatacatatccttttcaaaaaatcttaagtggggctcttgctatgcatactgttctgtaacttgttacttggattaacactgtatcttagacatctttctatgtagagcgtatagatcttccctgttcttttaaatggctgtataattgtctatggaaggacttaatttatttaacccataccttgttgatggcttatttgtgttttgcttttattttttcctctttgtttttgctgctacaagcaatgcttccttccatcttagcggatctgtctttgtacccttgaatgagaaagttgctggatcaaaggatgtattcattttgaattaggtgttgctaatttttcctccaatgatacactgatgtatcccccctgcccacagtgtgtggtcatgcctgttctctcaccctcttaccagtactggacattaataagcttttaaagatttgctactcaggctaaaagtgtctctttgttttagggtgcatttcctcatttaatgaagtgaagattcttccttgtttagtgaccatttgcctttatttttctgtgaactgcttgtgaatggcatttgtcgttcttctgttgtctttttagtcttttttctaaagcacactttgtagccctttgttgtaaaatgttggaaatatttttcccagtttgtcatttaatctttgactttgtctttctattccccagtaggaggtacttaatttttatatactcatatttggcaggctttttctttataggttcttttggctttaagtgatacttttaaacccagctattgctcatttaaattagaaccttttccatgagaaccacactgacgatttctttaaatatagcttgaaaaaatttttcccctattgttcttttagctattgttcttgaaaataatgtgttttttaaaggaatatctacaaatagaaatggtgatgatatccagcaaatgttttaaaatggtgtaaaaccatttgtactcctttagtaattttttggtaaaaaatttatactcctttagtaattatcatttttaaaatgatcagaggatgcattttttaactgttttattttttgaaagctcattgtttaacttattatatatgtattcatttctacagaattataaggctgtctgcagagatttgaaaaatggcaacaaatgaaagtgtcagcatctttagttcagcatccttggctgtggaatatgtagattcacttttacctgagaatcctctgcaagaaccatttaaaaatgcttggaactatatgttgaataattatacaaagttccagattgcaacatggggatcccttatagttcatgaagccctttatttcttattctgtttacctggatttttatttcaatttataccttatatgaaaaaatacaaaattcaaaaggtgagtataagggactagaaatagaatattatcattaatgttgctgaatattttaaaagtacatagggctttgttttgtgaggctaaagcagtgatatccaatagaaatatgaagccacgtatgtaattttaaattttctagtagaatacatagaaaaggtaaaaagaaataaggaaattaatttcataatgtgtatcatttagctcaataaatgtaaactatcgctgggtgcagggtccatgcctgtaattccagcactttgggaggccaaggcaggaggattgcttgaggccaggagttcaagaccatcctgggaaacatagcaagaccctgtctctacaaaaaagatacaaaaatacccaggcatggtgatgtaagtcctagctacttatgaggctgaagcagaaagattgcagcactatactctagcataggcgacagagtgagaccttgtctcaaaaaaaataagaaataaatgtaaattattatttcaatcagtaatcaaattctaaaaaatacttaatgagatatttaataagtctttgcaattccgtgtgtattttacattaattttagtctatctcaatttagactagccatgtttaaagtgtttggaagccacatgttactagttgctcctgaattgagcaacacagtcctaggtcattattgataacatttcaagaatactttgttaaattgggctttaagtagatgtgatggttatctaacttaagtttatgaattttaatgtttaagctagctggaaaggaaaggtgtggtgatttgcgcatattttgcagttcaccccaactctatgttccagtaaatctaagggactgttaatacactacgaccttgatcagggctattcaagttttttttccctaaatatatggtaggtagttctgcagcattcgtatcatcccaaataaggaggtgatgctcctcgtttctggatatttgcttcattgcactaaatgttgagaggtcgctatgtacatgacaaggtgaaatctcatatgtagcctgtgagcttgacgtgagaatttggagtagcttattagaaagatgaattatttgttagaatttgtaagctgatgatagtttctagtgtttgctgtttacttttcataaaaagtcattccaaactaaaactcaggggcacacagtcttggtagaaagtagaccattgagagtattcatctatggaaagtaatttacattcacttagtacaattggccctccatatccatgggttgttgtatccatggatccaaccaactgcagatcagaaatattcaggggaaaaaaattgtgtctacactgaacatgtacagtcttttttttccttgtcattattcaaaatgacaactatttatagagcatttgcattttattaagtattataagtgctgtagagatgatttaaagtatacgagaggattcgtgtaggttatgtcaaatactatgtcattttatatcaggcacttgagcatcttcagatcttggtatttgcagaaagtcccagaaccaatcctcaaaagataccaaaggacaactgtatatattttggatggcagtctgtacacattctctgttatcattctgttagtttcacagcctctcccagagtctcactttaagcaggtattaatattagtcctctctggggataatgcaggggtcagatgactgtggactccaggccaaaggagaaaagagcaaagggtaaaggcgaaggaaataaaaaataggagggccaaaggagagtactctgtgaccctcaattaaggtcacagaagctccaaagtgctttttaggaaagcagctgctttgaaaggcagaattaagtttggacgtctaagttctaatgcacctttagggtgattgtggctgccgtgtttcacccagtgatttatttatagggcttattcattgtaattcattgtatggctggccaggcaaaagcatcctttttctccttcactgcagtttgtaactgactcactggttagaagtagtaacctttgcagagagacaaaggactttctcaggcaagggtatatgagcagctttaaaatataatgtggcaaaggaaagaataagctgtagtctagttggtcagagctagttgtttatgaacagattgtaaggctggataatttgacttcaagtctgtactcagcaagtctttatgtttcataaccattaaagtccatgctttgagcatttttgataaaaaatgtgattttaaaccaggactagttttcacaagttaaaggagttttaaaagaaaccaaaatattggtacaaattaattacaggtttatgcatttcgaaggcagataccctgattaacattgagggtatcaattgtttaagataaaatatttgagaattatatttaacatatgcaataaatgtttttattcttaaaattgtcgaaaagaatagaagaagttggtggtggtgatgaaatagtactaaagactttctgctttcaaacagaacagacaactggagagctaatgcacatccttgctagttaggcgaaaatttcacaggaatgaaaaagtaaagcagactttgcaggatctatttctttaaaaaaaaaaaaaacatacatcttagtaattctccaaaaattttcctcaaagataaatgtactaaaaatattatttctgaagtttgtggcccttgtaaaggtattcctttatattaagtacagttatgcataaagaaagtaaaatatggtaaactttcatattgcactaggtatgaatttgtattgctaactgtctttgtaactaatttatgtatactgtaaatggtatagcatgtgattttattatagttgattaactttgtaatttctgtaactgcatcgatatcccagtctacctggaaaattaagtctattaaccatagttgctgtaggagacagtactattgccaactgaagcctgaatccttcatttattttgtccccaattacagagtggaggtttagaggagtggggttagataatgctcagattagaaatacaaaggcagctgtcagatcctcccattttattgttgaagaaactgagttgtaaacatcacaagagctagttaactggtgagtagcagccctggtattagagcacaagtctctggattgattcttagttcagtgcttttcctatttttgtcaggaagataacccttaaagaatttcaagaacagagctggatctggagacctagattttagttagtccaacttctgctaataactgcgtgtgtgaccctgcccaagctggttgacctctttgggcttctgctgatgcgcagtagttcccgtactttggatatcgtggttcaattaaaagagttttgttggcggatacctgaatttttcagcagtgacatttaaaacaaagcaataactgatatttattgtcaccatcgttttgttaagcccaaagcacttttttaagtgcagtcctataaattgaatacatttagttagtgtttgttttgttttgctttgttttttataatgacttgctaagcaaatgggtatcctgatgaggtcttaacgaacatcccatgttgatctaacttttctcattttgacttgaatctgtgaactccataatcaggacatatctgtgtacttctcaactcagagagtttataattctgtcattggatttgaacaaaagtgcatttatttgttggaatgaataccactgagtgcctggaagcatcgacttactgtgtaaaaggcttccaatgcttcgtatacaacttcttcaattgtggacacccaacagtaatcttagcatattatatttcttcttctctgaaacttctggtaaaagaagtgaagtgaatgatctgtggcagcaaagactggagaattattcattccatagtgtttcttagtttgtttgagatcatcatggctaggcgcatctgttaacagtttcttcacctgaagtagtgatagtagttgtcaagaatttagaaggcaaagattcctgagtcttagttatataaagttaacataactgacgtagaattaaggtccaacataaacagagaacaaattaggtcaagttaaactctgatagcagagactaatattagatattgtgatttttcttcgtaggataagccagagacatgggaaaaccaatggaagtgtttcaaagttcttctctttaatcacttctgtatccagctgcctttgatttgtggaacctattattttacagagtatttcaatattccttatgattgggaaagaatgccaagatggtacgtagataaaaatttggcttttacacccaattgtggcttattcagttaagttatacttaatgtttacccgttttcttaattttagttaatgtttgttctaaactttggaagtaaataaatagtagaaaagtaaaccacagtaaaatcttaaaatgtttccatttttacatcttttaaatattttattggaaggtgagcttctagtatcagaagtttccataacgtcttttgtatgtttatatacatgtataagtgcttatgttgacaaaaatatattacattttaattttaaaatgaatgaaatatatgagaatcatttatgaggtttatagaaattgtgtttacatgaacaaaaatatgtatgtgtatatatatatatatatatatatacacacatatatatatacacacacatatatatactcatgcgtcacttaacggatatctcttgagaaaagtgtcatgaggcaagttgtgtgaacattgtaatgaaatgaaattggtctaatgggcagtctctttaaccttatatcaagttatgtagctgtatctggtggttttgagaatttatttatgaatatatccaattaggtcaacctggtaagtgggtgggtggttttatgtaatgtctcaagcagtgatcccaactaaaagtctggatagtttaagtaaaaattatttcttacacattacaacatttttatcttaaaggtattttcttttggcaagatgctttggttgtgcagtcattgaagatacttggcactattttctgcatagactcttacaccacaaaagaatatacaagtatattcataaagttcatcatgagtttcaggtatgtgagagttatatttaattctttctgttagaggcaaaatgtctattttaattgcctgagcatttttctaaaattgttggtgacgtttttattttcttttcctttggcatgattattaagaacaatacacacacatacaaacaagccatttctacacattgttttcattatttaaatttcatggtaaattgagatctgaaagaaaaatattatatgaaagttcggacttccatccttgtggacagtgctacactggcacagctagatcctcacattgctaactcccacaaaaacagtaacttctatgagcactgctttttttttttttttttttttttttgagatagagttttgctcttgttgcccaggctggactgcaatggcatgatctcagctcactgcaaccttcacctcctgggttcaagcaattctcctgcctcagcctttcaggtagctgggattacaggcatgcgtcaccacgcgtggctaattttgtatttttagtagagacaggatttcactatgttggtcaggctggtctcgaactcctgacctcaggtgatccacccgccttggactcgcaaagtgctgggattacaggcgtgagccaccatgcccggccaattagaattgctttgatgtagctttgtcaactggttatgtgagtatgttttgcattgaccgtgattacatggtgtgccaaatcaagcctctctttattagaagaacaaatataaatacttaagtcaaaattagagttcaagtcaattatttaatgcctttatcttaaaccatcaaagacagcaagattttatatccctagacttttgatgtggagtaaggtatttttattgagaattgctagtattatttataagtgtatgactagataaatcatcactacatatagaatcaatataactttgtaaaactttatgcataaataggatatatatattagtgaagtctccagtgaagcagaatcattggggtatatatatgcagagagagatttattttaaggaatcagctcatgcaagtgtgcggctgtcaagtctgaaatctgtaaagcaggctacagactagaaatccaggtaagaattgttgcagccttgggtccaaattccatggagcagcaagttggaaactcaggcagggtttcagtgttgcagtctcgagaatccttcttcaggaaacctcagccttttatcctgaaggccttcaaatgattggatgaagcccaccctcattatgaagggtaatcacctttactcagtctactgatttaaatgttaacaacatctaaaaaataccttcacaacaacatctagactggtatttaatcaaacagttggatatcatagcctagccaagttgacacataaaattgaccatcacaatagctaagaaattaagaatttcttatctgtttgtcttaggctccatttggaatggaagctgaatatgcacatcctttggagactctaattcttggaactggatttttcattggaatcgtgcttttgtgtgatcatgtaattcttctttgggcatgggtgaccattcgtttattagaaactattgatgtccataggtgagtattaatttctgttcaggtataaagcataatgaaatatatttattttcatggccataagattatcatatttctaaggagactaataggagaagttaatcttcttaatgttatattaagaaaacataactgttggataaaagtttaaataatagatgtttttacattctagcctatgctgttataatttttatagtgataatgtgttattagggcaagtatatattcaggaccagcaatttccttatccttctgtaataaacctaaacttaactcatatttgaaaaaaatatcaaagcattcagccttccttgaataagactttctaatctctactgttcagcactgataaaggcacttgcaagatgaaactactacttgtaacacatacatatttcaaatgcatcctttctgttgattggaagacattttgtggtaaattatttatattgaatgccttcttaaatgcttatcctaattgttcattattttttaattatatgttcattgcattttgacttgggacatacttctgtactcatgaatgcagaatatcaaattctaagaattatttttaaagtgctaaagtagcaaaattaatgcttctagtcctaggcagagaatattcttctgtagaaaaattgtaattgacatttctttcttttttttttctatccattgtttctttctgccttccttcctctaagctcctcaaaggaagagagggttagagtgattcaaataagtataactggatgtctgattgtagatatgtagttggaaataaaggagcatactttaaatgggactcttttttgaagccatttgtcttctgccaactatagaaaagtacactggtattttgattaattgtggtacatttgattccaacttgtcattgcctaaaaaagtaaatgaagttgctatacagggattcatgggcctgccctttttaatacttgatactaattttatgtgacttttcctaaaaaacatatttagtattttgggctttatttacaactgttatacatgatggtgagaaagcttcctctaaaacataaaagaaaattaattcttaaaaatctgtgtctaaagattcattactataatccgtctcttccatcattcatatattttatcataaaataaatgattttcttagtttttttaaggattttttttcttagagtggtttctagaatatacaccattttctgtgtttgctgtttgtgaacacttagaaataaagtggtctaggcaaagtggcatgttatctaaattggttaatgtgaacacatgattattaataaaaacaacaatcatttgagatgtatttattccttaataatctttatcatttttgtttcagtggttatgatattcctctcaaccctttaaatctgatccctttctatgctggttctcggcatcatgatttccaccacatgaacttcattggaaactatgcttcaacatttacatggtgggatcgaatttttggaacagactctcagtataatgcctataatgaaaagaggaagaagtttgagaaaaagactgaataaatatctcacgtaaaccttcctgaaagataaacgttttcctgaattcagaaactagtagctaacattgcttctggagagcagaaataagcatgtcttctggctactaagtgataaaaagaacattaacaacctttaattaccttcctagtgggaactttttctactttacctacaagttctatatatgtagaaatgaataaatatatatttaagtacagttttcatgaggaagttttaaaagaccatgttcctaagcttccaagaaggttttggatactagaagtattaatctatggcttttctcccagtaaaaccataggcctgaagttcacattgggtctttaaatcttttagatatatactggtcatttcagaaaattcttcatagtggtattggccttatatttaactttttttttattttttttttgagacaaagccacactctgtctccttggctggagtgtggtggcacagtctcagctcactgcaacctctgcctcccagttcaagcaattcttctgcctcagcctcccaagtagctgggattacaggcacccgccaccacgcccagctaatttttgtatttttgtagagatggggtttcacgatgttggccaggctggtctcaaacttctgacctcaagtgatctgcccaccttggcctcccaaagtgctgggattacaggtgtaagccactgcgcccggcctttttaactttaaacatgttttagaattcacctaaagatcaaaatatcatggattgaacctcatcaattgatagcagtgagtgactgaagcttccaaatcaagaaaagccggcaccaagaacttccattctaatctagagctgaccagtttgagctgattctctctttgaagagtccttcttgattgcagtgcagtactggcatttctgaatggatgtaagtggagtattttagtctaaaggcttttcaaattacttgaatttttttaaaaattgaggagctttatttctatttacccttccatttttgtatatcaaatttccattgtcattaaaaactgtatcttgaaactttgtgaactgacttgctgtatttgcactttgagctcttgaaataaatgtgatttttgtgtgattatctggtttccagttttaaacattaactgtcaccttttattcttaaacttgaaagtacagaaatcattaaattattaagttgtacaataaaa